European Patent Specification EP 3 976 791 B1, published April 9, 2025. Title: COMPOUNDS AND METHODS FOR REDUCING FUS EXPRESSION. Applicant: Ionis Pharmaceuticals, Inc. The sequence listing filed with the application follows.

SEQUENCE LISTING (481 sequences)

SEQ ID NO: 1 - DNA, 5119 bp, Homo sapiens
acttaagcttcgacgcaggaggcggggctgctcagtcctccaggcgtcggtactcagcggtgttggaacttcgttgcttgcttgcctgtgcgcgcgtgcgcggacatggcctcaaacgattatacccaacaagcaacccaaagctatggggcctaccccacccagcccgggcagggctattcccagcagagcagtcagccctacggacagcagagttacagtggttatagccagtccacggacacttcaggctatggccagagcagctattcttcttatggccagagccagaacacaggctatggaactcagtcaactccccagggatatggctcgactggcggctatggcagtagccagagctcccaatcgtcttacgggcagcagtcctcctaccctggctatggccagcagccagctcccagcagcacctcgggaagttacggtagcagttctcagagcagcagctatgggcagccccagagtgggagctacagccagcagcctagctatggtggacagcagcaaagctatggacagcagcaaagctataatccccctcagggctatggacagcagaaccagtacaacagcagcagtggtggtggaggtggaggtggaggtggaggtaactatggccaagatcaatcctccatgagtagtggtggtggcagtggtggcggttatggcaatcaagaccagagtggtggaggtggcagcggtggctatggacagcaggaccgtggaggccgcggcaggggtggcagtggtggcggcggcggcggcggcggtggtggttacaaccgcagcagtggtggctatgaacccagaggtcgtggaggtggccgtggaggcagaggtggcatgggcggaagtgaccgtggtggcttcaataaatttggtggccctcgggaccaaggatcacgtcatgactccgaacaggataattcagacaacaacaccatctttgtgcaaggcctgggtgagaatgttacaattgagtctgtggctgattacttcaagcagattggtattattaagacaaacaagaaaacgggacagcccatgattaatttgtacacagacagggaaactggcaagctgaagggagaggcaacggtctcttttgatgacccaccttcagctaaagcagctattgactggtttgatggtaaagaattctccggaaatcctatcaaggtctcatttgctactcgccgggcagactttaatcggggtggtggcaatggtcgtggaggccgagggcgaggaggacccatgggccgtggaggctatggaggtggtggcagtggtggtggtggccgaggaggatttcccagtggaggtggtggcggtggaggacagcagcgagctggtgactggaagtgtcctaatcccacctgtgagaatatgaacttctcttggaggaatgaatgcaaccagtgtaaggcccctaaaccagatggcccaggagggggaccaggtggctctcacatggggggtaactacggggatgatcgtcgtggtggcagaggaggctatgatcgaggcggctaccggggccgcggcggggaccgtggaggcttccgagggggccggggtggtggggacagaggtggctttggccctggcaagatggattccaggggtgagcacagacaggatcgcagggagaggccgtattaattagcctggctccccaggttctggaacagctttttgtcctgtacccagtgttaccctcgttattttgtaaccttccaattcctgatcacccaagggtttttttgtgtcggactatgtaattgtaactatacctctggttcccattaaaagtgaccattttagttaaattttgttcctcttcccccttttcactttcctggaagatcgatgtcccgatcaggaaggtagagagttttcctgttcagattaccctgcccagcaggaactggaatacagtgttcggggagaaggccaaatgatatccttgagagcagagattaaacttttctgtcatggggaaagttggtgtataaatgagaaatgaagaacatgggatgtcatgagtgttggcctaaatttgcccagctatggggaatttttcctttaccacatttatttgcatactggtcttagtttatttgcagcagtttatccctttttaagaactctttgatcttttggcccttttaatggtgaggctcaaacaaactacatttaaatggggcagtattcagatttgaccatggtggagagcgcttagccactctgggtctttcacaggaaggagagtaactgagtgctgcaggagtttgtggagtggagtcaggatctaggaggtgagtgactcccttcctagctgccctggtgaacagcgcttgggtagatacctgctataaggagactggtctggctgggttactttcacatcctgcctgtactcagagggcttgaggtcattgacattatgagattttaggcttgatccctttttgattggagggtggaaggccctcctaagggaatgataagtgataagagggggaaggggttgcagccaatgagttaaaaccttagagcagtgctcctcagcctcttaccatgtggttgtaaacttgcacgtacctgccaaccagttatttagcatgctttttattttagttacacagagcgtaacattaacccaagagcagaaaggttttatttacagggttttcgaacttggtttgtaagacagctgccatcacaagcatagcttacaaatgtgctggggacccctaattgggaagtgctttcctctcaaatttttattttttatttttagagacagagtcttgctctgtcatccaggctggagtgcagtggcgtgatctcggctcactgtagcctctgcctcctgagtttaagcgattctcctgcctcaggagaatcccagcttctgagtagctgagactacaggcgtgggccaccatgcccacctagtttttgcatttttagtggaggtgtggtttcactgtgttggccaggctggtctcttaactcctgacctcaggtgatccacctgccttggcctcccaaagtgctggaattacaggcatgagccgctgcatctggccatcctctcaaattttcaagtgttccacaagtatgttctctactgaagagttgctgcatccttgaatcttgggtgatttgaggcacagaaactatgactttattttttgagatggagttttgctcttgttgcccaggctggagtgcaatggcacgtttttcggcttaccgcaactgccgcctcctgggttcaagcgatagctgggattacaggcatgcgccaccatgcccagctaatttatttgtatttttagtagagacggggtttctccatgttggtcaggctggtctcgaactcccgacctcaggtgatgtgcacacctcagcctcccaataaaccatgacttttaagaggaatagcaggtttacttcccctgccagcattggggtgctctctaagcaacagtaggcggagagtggtctggcgtattaaaaacaaaggatcgtcaagtgggccttcccaggcattgctttgacttagtacatgtagaggatgtggcagttctctccgtccctgccactgctggtttctttgttaaatgtttagttgaaatggcctgatacgatatttgagtagttcactgttggtgctttgcctagcaggattctaatcttgctttggttgtggtcccctgatgccctcctgttaggagtggaggaggtcgaagctccttgtaagatatgattactgggaccattagtgtcaagttcctgtgtccttcaaatggcatatgtgattggccttgaccttaaaaggaaatagggtcccaggtgactgtttagtgggtaggtccagtttggggggatcttccaggagaatggatagagacacctagcagcagagagaacattggtgcctctcaagccaacctcccacctcagcctcccaagtagctgggactacaggtgcttcctcgctaccacacctgggtaattttttttttaattacttttttttttttaagaaacagggtttcactgggttgcccaggctggtcttgaactggcctcaagtgacctgcctgcctcagcctcccaaagtgctgggatcacaggtgtgacccactgcgtttggccagaatactctattcttactgaatgattgaaatctgtcttgaagcattaggtgtcccatttttgtgagttggaattgggacaggctaagtaggaagtgaggagggtggggagagctgtgctgtaggtctgtttgtcccttccttgatgtagccttcagttagccctttcagcttttttccccatcttgtgccgggccttcctgggtttcagtacttggatgtagggctgcagttatgtcagtggtgggtagattgaccaggaattaaggtctagggtccagcccatgtgagacttgactcactgatctacctttaggcatgtcttccttccagtctcatcctttttaaattttttttttttttttgagacggtctcactctcacccaggctggattgcagtggtgtgatctcgaccaactgcaacctctgcctcccacccgcaagctatctgcccacctcagcctctggagtagctgggacgggactacaggcacctgccaccatgactggctaatttttttttgtattttttgtggagatggggtcttgccatgttgctcaggctggtctggtctcaaaactgctctgggctcaagtgattgtcccactttggcctcccagagtgctgggattaaggtgtgagatactgtgtccggctatgaaaattttatttttaattaacttgtatatatttatggggtacaatgtcctatttctgtacatgtacacattgtggaatcaaatcaggctaatatatccatcacttcatatcattagcatgaatgagaacatacaaagccactcttagaaaattttgaaatttatgttatttcagcccttttatgctggaggttgcaaatgttttgtgaataatcagaccaaaaataaaaacaaaaaatgattgacttcagtcattcagtaagaa

SEQ ID NO: 2 - DNA, 22000 bp, Homo sapiens
ccagcctgggtgacagagtgagactctgtctcaaaaaaaaatcaatatctgatatacgtgtttatttttttattgagatggagtcttgctctgtcgcccaggctggagtgcaatggcacaatctctgctcaccgcaacctctgcctccctggctcaagcaattctcctgcctcaacctcccgagtagctgggactacagatgcgcgccaccatgcccggccaatttctgtatctctagtagagatggggtttcaccaggtcggtcaggctggtctcgaactcctgacctcatgatctgcccacctcagcctcccaaagtgctgggattacaggtgtgagcgaacgcatctggcccaatatctgatatacatgttaattgaaactgggtgtggtggtcacacctttaatcacagcactttgggaggattcccttgagcctaggagttcaagaccagcctgggcaacatagcaagaccctgtctcaaaaaagaaaaatttaacattgactttcctgtcagagataggaagtaaataagacatttatggtgaacttaaagcacatatggcagctaaaggtgacagtgtctcactccagctgacccttgccctatggaagtgggcctggaatggcccactatttttagtgttggcaactagttaaaaaaattaaaacattcgaggcaggtggatcacttgagatcaggagttcgagaacagcctgggcaatatggtgaaaccccgtctctactaaaaataggaaaattagctggacatggtgatgcatgcctgtaatctcagctactcgggaggctgcagcacaagaattgcttgaacccgggaggcagaggttgcagtgagctgagatcacgtcactgcactccagcctgggtgacagagtgagactccatctcaaaaaaaaaaaaaaaagaaagaaagaaatggccatttgatttagtctttcagagtcacatatttttttttttttgaggccgagtctcatctgccaccatgcccagcccagagtcacagctggagcctgaactctgcctcagtgtcttccccacttgtgcctttgtcttcgcggttctgcctattatagcctttcctcccttgctgcttggcaaacttctacttatccagtaagccttggcttcagggttaccatctctctttagtgttctgtggttgtccacctgatggatgacttactctgctggcagggtttccagtctttgattccatgtgatggcacttactacactcaagtacactttgtggtctgtgtgtctcacccacattcacccactggctggtcctgtggtttaggaactgagcttttttttatccatatccatccagtcggccccatgattggaacatactatgcagtgctcaggcaatgtttgctgaagcgcaggggttaagagcaggctacctggcttgggaacccagctttgccacttcctgtgtagcttcagcataactttccgtctttctttttttttagagacagagtcttgctctactctatcatccaggctgcagtgcagtggcgcgatctcggctcactgcaacctctgcctccggggttcaagcaattctcctgcctcagcctcctgagtagctgggactacaggtgcgcgccactatgcctggctaatgtttgtatttttagtagagacggggtttcaccatgttggtcaggctggtctcgaactcctgacgttgtgatctgccctccttggcctcccaaagtgctgggattacaggcgtgagccaccgtgcccggtcaactgcctgtctttctatgcttatttcctcatctgtaaaatgtcatccttagcagggcgtggtggctcacacctgtaattccagcaatttgggaggccaaggcagatggatcatctgaggccaggagttcgagaccagcctggccaacatggtgaaaccccgtctctactaagaatacaaacattagctgggtgtggtggcgcacacctgtactcccagctacttgggaggttgaagttgtagaatcacttgaacgcgggaggcacatgttgcagtgagccgagacggcgcccctgcactccagcctgggtgacagagtgagacagtgtccccccaaaaaaaaaaaagataaaatgtcatcctcacatcagccttttgttgtgaaaaataaaatcaagagtttactcagtcagaacagggcctgacagtaagtcttgttaaagtgttagctattacatattatagatgagcacaatgtatatcattattaaatgtcagctttattattattatttgttttgagacagtcttgctctgttgcccaggctggagtgcagtggcacgtcttggctcactgcaacttccgcctcctgggttcaagcgattctcccatctcagcttcctgagtagctgggattacagatgcgcggacgacgcctggctaatttttgtatttttagtagagacggggtttcaccatgttggccaggctggtctcgaactcctgacctcgtgatccacacgcctcggcctcccaaagtgctggtattacaggcgtgagccaccgcacccggtcagctttattattaaatgttaacttcatctgctttgtacacgaatgcatacccagtgcccagaacagtgcctggaacatactaggtgctaaataaatatttgtgacttaatgcatgaataagggtggacttcctttcttttgctctcactggagagttgaactctccttccaaaggcggtggggtggatattggcatattcagggcctttagggctgaagtcaagggcttagtggggcttaatttgtgggcgggcccagggcatggccctcattgtttctctagaaagacgtgtccaaccctcaaaggaccttctgaaatcccgctgaaaggttaagttgggaaggaaaacctgcatgcctatgtatcaggaattaacgtcttttgtcttgttttattcagtagtttcaaattgccttctccaggcaaggctgatgaaagtgcaagttgcaagttaatttgaatgtttctttttgcttttgctctcacaggaagtgaaaaggcgaccaaacactctagcattcatgccaccaaaaagaggagtgttttgcagttacaagacctggattcgaatcacgactcctcttagctgccctgtaatcaggcacaattacttgggtctctgagtctcactttccttatctagaaaacggaggtatctttacttccttcgtaagactgatgacaaggaaattatctgtgcattttgaaaccacttaagccttgtacacgttttatttctgggatcgccctggtagggcttcagaaaaataaaaaggaggtccctgagaaaaggctgggtaccgtacatctgaggtcaaccctctctggtcccaaggatggcctgggctgttccgccccgtggctccccaggggcaaagccatgaggatccgggtgagagcccagtgctggacgagcccggggcccaggggtcccggccgaaatccctgctgtctttcaggtcaaacgtcataatccccgaaccccagaaaggccgaaaggcaaggcaaccctgaaagacgacgaagtcaacctcagggcgcaggagagggagggccagtgtgctgccgacgagggaggctggagccgcggggacgaggcgccccatacagcggcaagagggtggagggcaggagctcgccatcctgggtgaaagcggggcccagcgaaggggcccggccacaggaatctcggttccaccccgctactcccggctgtgactccagtttcgtccccagccgccgggaccgccccctcgccccgcccccagcgggcactcaggccgtaccactgtgccttcatgggggtggagatagatcgtgggctagtcctgccgaggagagaggggttcttcctcaaaaaatatgattatgtatagtattcgcatgattctagttaacttgtttcccttctgcctgctcggaccctctacctgccctacgaagggggcggagtgcgttcctgcctccccctgctcttccgcgtttggtgcgcgcctgcgcggtgcgtaggcggcggagcgtacttaagcttcgacgcaggaggcggggctgctcagtcctccaggcgtcggtactcagcggtgttggaacttcgttgcttgcttgcctgtgcgcgcgtgcgcggacatggcctcaaacggtaggtaagggcgcgaggcgacggcggcggcgcacccggccgaggcctcccagctgggcttttcgttttcagtgggaccggggcggcgatcccgtgtgggattttttggcgcccctgtggcgggaagccgcggagaagagtaactggaggaggctggtgtcgccattttgtttcgctcctctggccctcgcgcgcggggcgggaagtcttttctttgcagtccgtttgcttggggtgggcgttgggagggacgcttcttaggggtttgaagcgtcaggtgagggtggaaaacgcccattctccgtggcctcgcctcccccaactcccggccccgcgctcgagcccgctttgtcgcagtgctgcatccgggcactcgcggcgcgcacgcgctctgcgggcccctcccccttcgcggcgcgggtaccccttccccgcctcgtgttggttcagctttctgtcgcgagacccttcgcggaagactcggcggcgcgcgtccggtgtgagccttgtccctcagtggtccttcgcgaatgggcgggatcgctccgttcccgcctgggttgccacgcggctgggggcggaggctcgggatcggggccgccctctagcttaacggtttggcggcggtggtcagggttcgaccaacggacttggggacggcccgagagtttttcccgcctaaatttctttctttttttttttggagacacggtcttcctctgtcgcccaggctggagtgcagtggtgcgatctcagatcactgcaacgtccacctcctgggttcaagtgattcttctgcctcagcctcctgagtagttgggattataggcgcccgccaccacagcccggctaatttttgtgtttcttagtaggggcggggtttcaccatgttggtcaggctggtctcgaactgctgacctcaggtgatccgcccgcctgggcctcccgaagtgtcgggattacagacgtaagccaaccacgcctggtctaaatttcttttttctgagatagggacggagaagaacggccgcccgaggccacaccctctcctggtcctctttcccttttcctgcgggggaagcgccgcgtttcctgtgctgggaggatgagttgatcttgttcgtgtatcttaagtggggcttttcaaaagcgcttttgttgctttttgttcgctgggggaaggcagggtaggtgagaaaacggaaccatctggagtcccagggctggggactcgagtacctgttgactttcgcctcctaaggcgagcagttgcatgatctctgtcatttggggtccaagggctcttttgattctctggctttgcactaaaaagcccacttcatctccgggattggtcaaagagtgaagaatggccttttttgagactttcttattctgtgggtctgggctgagagagcagaggccacaatctgaacactgttcgaattcaaacctgtgccactttggtagttctgcgacgttgggagagttagtctcttgactcctggcgataatggctttctcatagagtggatgaaacgaatgcgcgatgttttagagcaatcactgacatgaattgggcttgcagaaaattgtggatgtccaccaagaccttggtttttccaatggttaaggcttctgggactctgtagaaacttgcattttcttcactttttctttattgtaagaacacttggctgataacgccagtttgttcctcttctcaaccagtgtctcatggaggaattttatgccctttgttgcaacatggtcctatttttatttttttttttgagatggagtcttgctctgttgccaggctggagtgcaatggctcactgcaacctctgcctcccgggttcaagcgattctcctgcttcacctcccgagtagctgggattacaggcgtgcgccaccatgcccggctaattttttgtatttttattagagatggggcttcaccatgttggtcaggccagtctcgaattcctgacctcaagtgatccacccacctcggcctcccaaactgctgggattacaggcatgatccaccgtgcctggcctacgtggtcctttttattcatcagtgcttgagttaaggaatttagctttaattcaactctttcagagtggcagctgaagataatgtgattgtatttttcttttgcagattatacccaacaagcaacccaaaggtgagtgctatttttgggcttccagagtttgtagagggcaagggtggtcacgccatgttttctgatcacgctggttttccttttatttagctatggggcctaccccacccagcccgggcagggctattcccagcagagcagtcagccctacggacagcagagttacagtggttatagccagtccacggacacttcaggctatggccagagcagctattcttcttatggccagagccagaacagtgagtctttctcagcgggtcacctcttcctactctttctgaatattgcttttctttttcttgttttttggagacggagtctggtcctgttgcccaggctggagtgcagtggtgctgtctcagctcactgcaacatcagcctaccgggttcaaacgattctcctgcctcagcctcctgagtagctgggattacaggtacctgctaccacgcctggctaattttgtgtttttagtagagatggggtttcaccgtgttggacaggctggtctggaactcctgacctcctgcctgccttgacctgccaaagtgctgggattacaggcgtcagccacaatgccctgaatgttgcttttcttaaacctgagcagcactgagatgttgaaactgttccatatttcttttccgtgaaacagtgtataagtcttaaaactttttgggatctgagtcctttacagggcattgtggcacacctgtagtcccagctactgaggaggctgaggcgggaggatcccttgaattcaggagtttggggctgcagtgagctatgatggtgcctgtgaacagccactgcattccagcctgggcagtgtgttgaggccccatctcaaaaacataaaaaaaaaaacaaaaaacaaaaatgtttattggtttgtgattctgtttccatttattttctttggcttttaatttttttgactcttcttattttccatcagcatgaaagagagcatattttctaaaggaagaaccagttttaggccaattctgaaatggagaaaatggttttgtttgaaaatgtatgaaatcatgtgatacataaggaggtgggatttgccccaaggtcctgaagtgtaactaagaaaggtggttgtcctgtagatactgcacgcacagctgcatattacagtgctgttaacagggatccttgggcctgggtttagagggtggtgctggagatggtgttgggattggcggggtgaaattggaactgtactaaagagttggtagaagttgaagcattaaatttaggctttgaaaggagggtaactatctttgcctatgagttgcaacatcactaacagcttctgagaggctggctttatgagtataggtattatgttttctttaacccattccttacattttctctttcctggtggcttttgtgactccctttttcttatcctggtagcaggctatggaactcagtcaactccccagggatatggctcgactggcggctatggcagtagccagagctcccaatcgtcttacgggcagcagtcctcctaccctggctatggccagcagccagctcccagcagcacctcgggaaggtacggtggtgttgatgtcggggaaggcttgaaaagaggggtgaattgatgaggaatgataaagggaccagcagtaggagcagttcagaggtgtaattggggtaggggagcctgtgttgggtacagagaatggactccactaaaagtgaaaggaaattgggggctatgctgggattgtgattgtgttttttgtttgttttccctagttacggtagcagttctcagagcagcagctatgggcagccccagagtgggagctacagccagcagcctagctatggtggacagcagcaaagctatggacagcagcaaagctataatccccctcagggctatggacagcagaaccagtacaacagcagcagtggtggtggaggtggaggtggaggtggaggtgagatgtcttcagctttgtctgcagcccattttctttttctttttttttttttttttgagacggagtcttgctctgtctctgttgctgaggctggagtgcagtggcacaatctcggctcactgcaagctccgccttccgggttcgcgccagtctcctgcctcagcctcccgagtagctgggactacaggcatccgccaccacgcccggctaattttttgtatttttagtagagacggggtttcaccatgttagccaggatggtttcgatctcctgaccttgtgatccgcccgccttggcctcccaaagtgctgggattacaggcgtgagccactgtgcctggtgtctgcagcccattttctataaggatttgtattctcctgttttagcttaaaagagggttcctgtcttgtttcctagctgtctttttactttcttttgtccttcattgcctggcacttgtcaaaccttttcaaaccttttagtgctactttacaatctttttgttttttttttttaatcattctttcttttctcacaggtaactatggccaagatcaatcctccatgagtagtggtggtggcagtggtggcggttatggcaatcaagaccagagtggtggaggtggcagcggtggctatggacagcaggaccgtggaggccgcggcaggggtggcagtggtggcggcggcggcggcggcggtggtggttacaaccgcagcagtggtggctatgaacccagaggtcgtggaggtggccgtggaggcagaggtggcatggggtaggtgtctcatgagccagggagtatctttggtggggagtgtggaggattgcatgaatctccctgaagccagtccctagtgcatggtttagtattcttgttgtctagggatctgtgagggctttgatttgggggcagtgactttctttttacatccccattttatttttgtgagaacttgggagcctgaactcccatccataccactgaatagagattttgagtaatgatacttgtttccaaaaaaaaagaaaccatacatagatacgtatggattggagtcattaatatcctaggcaagaaacatggaagtgaagacttctttctctgcaagggaaaccgatgatcccactcctgggaaatagtagggaaacttggtatgtgtattcccatgtgtcctctagggagttggtaatggttaacctgacttcagcttccaggaattggctactcttcccgttttctatagtcatttgaatccacgagcttgatttgcactaatttgaccgacattgattttgtgtgtgacttggtttatggggccagctgactgaagtaagcagaccttttgggcaaaaatatgctttgacagtggtctcccacctatttgttccactgtctgccttcccctggttacttaaaattcatcagcttgtccaactggaccttctttccttcctgctgaagttgatttgaagtaaaaccttagatttgatgttaaaacagttgtcaaatctgttggtaaataagatttgaaggaccctactctgtctcccttgaaaaaggggaggaatgtcagtgttactgtttttggaaaaagtagatttttaaaccgagtttggaaatggtaagtatgcagaggtgggtgggggcaatctcaaaaacgtgcaaaaatgaggaaaacaaaaatgaggaaatgtgtgcgtgtgtttaatgcaaaactttaaaaagaaaaacaactgttatgtgactgttaacttgctctgcattttatgtgccacaggtatgaaaggtgacattgcaaaatactccgctcttctcgcagtgtagaaggggtgaccccgggggttgggggagatcaaaaacagctcagtagttaggacagagcttagctaagtttgtcttgctttaaggggaagttgcctttggttttgactttttatggaatggggttgggtctgcttgctgctttcaaagcaaaaaccacaaaaatgtgttcaaggctaccccagcctggtgtgaaatgtcttctgggtaaattggggtagggtttttaaaccaactacttggttgtcaaccacttgcgacaagaggaaaaaaaaacatctgctccatcggaagaacgaccaaggaaaatgggttattttttttccagaggaaatagataacgtaaccttttaaagcaaaatctttataaactgtgtctgagaaattgcacacgtgtgtgtgacatgctcaaaggtcagacaaggggtggtcaggaagggatgtattttagtagccacttgtatctttttccaaaaacacctacccatgtttggggaatgttaaacaaaatcaaaaaacaaccttttgtagccgttggaagcttcatgtcctttcttctaacttgtcttctccagcggaagtgaccgtggtggcttcaataaatttggtggtaagtgaacagagtttccaaaattcccaactcccagcaatgctttgtctgattgttcatttgcagatgtcttagcgtgttaatttaaatgtcaaaggttttgaggtgtccagaaccacctccagaaaggggtagggtagaatgccacctgttgcctggtgtgtgctaacctggagcaggtaggggtaagactcaatagtcatcttttaccaaatgggtttgccccaggttaataagaggggtctagtaggccttggactgggccgttgccacacctggcacttagtgaccatcatcatgagaaactggagagtgcgtgctggaacacgtggtgccatcttggctttaggatccttttgatcgttgtgtccaaggcttgtgtgtgtgtgagtgtgtgggagacaactccgaatgtttaattctggaagagggatgtaacattgccctgaggatggtgaagttggtatacatttataaagtacggaatggtgtcaatgaatgcaattctatgtatatggacttaactgagatgggcaaatagaaactagctctgggaaggaacatgtgcactacttcaagaaagattggaagcatgtgtggctcatgggaaataaccaggtcttaaacagcacaaactgaattcgtggaccaggaaggtcttaaacagcacaaactgaattcatggaaaaatgacaaatttgagaagtctcccagtaagctggaacttttctggtttggttaacaaaaggtttcttgatttgtttcaagatttaaagccaaaggtgtgggttcatgacttaggtgtcattgcgtgtgggtacaatatttatatatggcgaattcagataaacattggtcaaagatggtctctggaaaaacaaaatagaggctgcattacggaaataagatttctggtctgttccctgggacatgcttaaaaaatacaatagctattatgtatggtttttattttcatgtggtttcggggaaacaacacggttttaaggatggtttctaaagatgaaattaaaaattgttccacaagggttaagtgtctggtggtaaagttgggagaaactggatggatgcacatcgcatggctggtggcgagcccatctctcttctctcgggtgagagaaccgggccaagctgagttggtttgttcactttaatgggtctccgtttcccctgccacctgtgctgaggacatttcccagcctgagctgggggaggcagcatttgctgaagtgtggagttgtctctgtggagactcaagttacagatcttaaggggcctgcctagaattttctcctctgggcaggcgacccaggaaagggtttggagtgaggctgtgagcacttacttgatattttacaagtttggatttggtgttaatttttttccttgtccgttttttcctgttgactaacggctcatcttttccttgtttttgttttttttttgttctttttttccatgtcactaaaggccctcgggaccaaggatcacgtcatgactccggtgagttcacacgtggtggcatgaaaagagtggctaaagtggtatcaagactgcctggatgttctttgaaactattataaaaaggaaactgaaaaaaatggggatagagaaggaagggagttaggtgtgtccttagttagcagtgagaagtatttgttacgaagtatttctcagaaatacctggcttgtgggttccacccccagtgatttaggtctgagaggaccctgaaaatctacctttctaacaagtccccagtgatgctgatgcgtctggaccacactcagatggtttacagcagtggttctttcaaaatgtggatcatgtccaagttggtgaacaaaactagtgaaagacctgaccacatgaagtaaagcattgaactcctgtttaggttgtattgatgtttgtgtactagatttgaatgtaaaatgggtttcttatttaattcggggaccttcaactgaaagttgataaatactgatggacttttctgtgtggtcttgttgggcatttcactcctgagccctggtttccatactgtatactgggtgttaacatgtttcaaaggataattgtcaaactgaatctgaaatttatcagcatggctggcatatagggactcaaaagggatgtggatttctttttagttgtcttccataaaccaaatgataccagttgcttgatggatactaggtgctttaggttttttcctgtgttttttattttaccttttcacatttgcattttctctgttcaacaagcagaacaggataattcagacaacaacaccatctttgtgcaaggcctgggtgagaatgttacaattgagtctgtggctgattacttcaagcagattggtattattaaggtacttgtggagaggagtgggagctttctgtcagtgttgtaggcttgtggatttcacacattagtaaaagcaagtctttaatggttgccagcagtaaaaacaagtcttagtggttgttgccagcttaatttgttgaggaaagagccttagttactgttttctaaaagagaagttctatcttaacacaaaaagtataacttatcagagtaccctaaactcttgagatttgtactctatagtaacttttagttttatctttcaatattggagtgagagacagttttctttaatggaggtttacatgtgaggtaggaagaagtaactgggaagaggggagctgaagtttgggaattataaacctcatgttctagaggaagaagatggaaagggagtactgtagcctttaaaattgatgttacctcattttgctttcttcagacaaacaagaaaacgggacagcccatgattaatttgtacacagacagggaaactggcaagctgaagggagaggcaacggtctcttttgatgacccaccttcagctaaagcagctattgactggtttgatggtatgtatgagaaggctggcagaggtggggctggggatatagggcagcaagccttaggaaacaagccatagtttgagggttcttttgagtcttccaacacttactttagctgcggtttcaggtagtctcatttttgcttatgtgtcagcagattataaaccatttgagaaaggcacgcttctcttgtattttcggattaatgtgtcttgcatttaaagtctgttgatgattttttgtttctctaggtaaagaattctccggaaatcctatcaaggtctcatttgctactcgccgggcagactttaatcggggtggtggcaatggtcgtggaggccgagggcgaggaggtgaggagctacctgctagtggtgcagaggggtaatggggagagtgcagaagatggtaaaggcttgcatggaatgggttagatttaccaaacttggagagggagcagacccatacttggtctatctgcattaggacccatgggccgtggaggctatggaggtggtggcagtggtggtggtggccgaggaggatttcccagtggaggtggtggcggtggaggacagcagcgagctggtgactggaagtgtcctaatccgtgagtgaaacttaatttttttcttagttctcttgcatgcgtgctctttgatatattggtactgaggtatgtgcgtgttttccaaagaagtaaatgtcaaggccacactgttggggtcagatttagccaaaagcttacctaggtaaggttgatgtaatgggaaaggtaatggattgggttcagtaatactgatttttgttcctgactctgagaagcaagccgttttgtctttctgaagcttcagtttcctcactgtatctctaaagtcaccgtagtttcttcctagttctaggtcttgcctattccccatcgctccagactgattgtcttcctttctccttagcacctgtgagaatatgaacttctcttggaggaatgaatgcaaccagtgtaaggcccctaaaccagatggcccaggagggggaccaggtggctctcacatgggtaagaaaggcagacctggtgctagggagctgggaccaaagaatccttaatttttcagcggggaggctcggggaacataggggaatgggaatatgatagatcttgtttcttttgtcctagggggtaactacggggatgatcgtcgtggtggcagaggaggctatgatcgaggcggctaccggggccgcggcggggaccgtggaggcttccgagggggccggggtggtggggacagaggtggctttggccctggcaagatggattccaggtaagactttaaatcagaataaaaaagtagagcagttgaacagaggccataggataacagggttttgttgagaaagtggtttcattttgagggctaggtggaaagacctgaggttgtaaccagtagtggagagggaaggaaaattaactcagggggagtgaatctgtagacccacttgagataagatactcgctgggttaggtaggaggggcagataggatatctaggcttggagaggctggtaactcaaatataatggatacttaatttttttttttttttttgcaggggtgagcacagacaggatcgcagggagaggccgtattaattagcctggctccccaggttctggaacagctttttgtcctgtacccagtgttaccctcgttattttgtaaccttccaattcctgatcacccaagggtttttttgtgtcggactatgtaattgtaactatacctctggttcccattaaaagtgaccattttagttaaattttgttcctcttcccccttttcactttcctggaagatcgatgtcccgatcaggaaggtagagagttttcctgttcagattaccctgcccagcaggaactggaatacagtgttcggggagaaggccaaatgatatccttgagagcagagattaaacttttctgtcatggggaaagttggtgtataaatgagaaatgaagaacatgggatgtcatgagtgttggcctaaatttgcccagctatggggaatttttcctttaccacatttatttgcatactggtcttagtttatttgcagcagtttatccctttttaagaactctttgatcttttggcccttttaatggtgaggctcaaacaaactacatttaaatggggcagtattcagatttgaccatggtggagagcgcttagccactctgggtctttcacaggaaggagagtaactgagtgctgcaggagtttgtggagtggagtcaggatctaggaggtgagtgactcccttcctagctgccctggtgaacagcgcttgggtagatacctgctataaggagactggtctggctgggttactttcacatcctgcctgtactcagagggcttgaggtcattgacattatgagattttaggcttgatccctttttgattggagggtggaaggccctcctaagggaatgataagtgataagagggggaaggggttgcagccaatgagttaaaaccttagagcagtgctcctcagcctcttaccatgtggttgtaaacttgcacgtacctgccaaccagttatttagcatgctttttattttagttacacagagcgtaacattaacccaagagcagaaaggttttatttacagggttttcgaacttggtttgtaagacagctgccatcacaagcatagcttacaaatgtgctggggacccctaattgggaagtgctttcctctcaaatttttattttttatttttagagacagagtcttgctctgtcatccaggctggagtgcagtggcgtgatctcggctcactgtagcctctgcctcctgagtttaagcgattctcctgcctcaggagaatcccagcttctgagtagctgagactacaggcgtgggccaccatgcccacctagtttttgcatttttagtggaggtgtggtttcactgtgttggccaggctggtctcttaactcctgacctcaggtgatccacctgccttggcctcccaaagtgctggaattacaggcatgagccgctgcatctggccatcctctcaaattttcaagtgttccacaagtatgttctctactgaagagttgctgcatccttgaatcttgggtgatttgaggcacagaaactatgactttattttttgagatggagttttgctcttgttgcccaggctggagtgcaatggcacgtttttcggcttaccgcaactgccgcctcctgggttcaagcgatagctgggattacaggcatgcgccaccatgcccagctaatttatttgtatttttagtagagacggggtttctccatgttggtcaggctggtctcgaactcccgacctcaggtgatgtgcacacctcagcctcccaataaaccatgacttttaagaggaatagcaggtttacttcccctgccagcattggggtgctctctaagcaacagtaggcggagagtggtctggcgtattaaaaacaaaggatcgtcaagtgggccttcccaggcattgctttgacttagtacatgtagaggatgtggcagttctctccgtccctgccactgctggtttctttgttaaatgtttagttgaaatggcctgatacgatatttgagtagttcactgttggtgctttgcctagcaggattctaatcttgctttggttgtggtcccctgatgccctcctgttaggagtggaggaggtcgaagctccttgtaagatatgattactgggaccattagtgtcaagttcctgtgtccttcaaatggcatatgtgattggccttgaccttaaaaggaaatagggtcccaggtgactgtttagtgggtaggtccagtttggggggatcttccaggagaatggatagagacacctagcagcagagagaacattggtgcctctcaagccaacctcccacctcagcctcccaagtagctgggactacaggtgcttcctcgctaccacacctgggtaattttttttttaattacttttttttttttaagaaacagggtttcactgggttgcccaggctggtcttgaactggcctcaagtgacctgcctgcctcagcctcccaaagtgctgggatcacaggtgtgacccactgcgtttggccagaatactctattcttactgaatgattgaaatctgtcttgaagcattaggtgtcccatttttgtgagttggaattgggacaggctaagtaggaagtgaggagggtggggagagctgtgctgtaggtctgtttgtcccttccttgatgtagccttcagttagccctttcagcttttttccccatcttgtgccgggccttcctgggtttcagtacttggatgtagggctgcagttatgtcagtggtgggtagattgaccaggaattaaggtctagggtccagcccatgtgagacttgactcactgatctacctttaggcatgtcttccttccagtctcatcctttttaaattttttttttttttttgagacggtctcactctcacccaggctggattgcagtggtgtgatctcgaccaactgcaacctctgcctcccacccgcaagctatctgcccacctcagcctctggagtagctgggacgggactacaggcacctgccaccatgactggctaatttttttttgtattttttgtggagatggggtcttgccatgttgctcaggctggtctggtctcaaaactgctctgggctcaagtgattgtcccactttggcctcccagagtgctgggattaaggtgtgagatactgtgtccggctatgaaaattttatttttaattaacttgtatatatttatggggtacaatgtcctatttctgtacatgtacacattgtggaatcaaatcaggctaatatatccatcacttcatatcattagcatgaatgagaacatacaaagccactcttagaaaattttgaaatttatgttatttcagcccttttatgctggaggttgcaaatgttttgtgaataatcagaccaaaaataaaaacaaaaaatgattgacttcagtcattcagtaagaatagtgtgttctggccgagtgtggtgggtcacacctgtaatggagcactaggcgtaaatgggttgaaacgggtctccctatgttgctcaggctggacttgaactcctgggcttaagtgatcttcttgcccttagcctctcagctgggactatggatgcatgccactgtgtctcacgtttttatgaactgtagtcaccatgctgtgcagtggcttaccagaactcatttcttgcatctgaagtgttgtaccctttgtctccctgcttacccatacctccaagcctctggtaacccccattctactttcagtttccgagtttgactttctagattccgtgtataagttcatgcagtctttctgtggcttattttagcataatgtcttctagatttatcgattcacccatgttacaaataacggtttccttttaaaaagctgaatagcattctgttgtgtctacataccacatttaaaaatccatccgttaattgggcacttgggttgcttgcatatcttggctagtgtgaataacgctgcattgggtgggagtgcagacatctctgacgtacagatttcttttttcttttttggagacagagtcttgccctgccacccaggctggagtgcagtggtaggatcttggctcactgcaacctctgccttccagattcaagtgattctcctgccttagcctcccaggtagctgggattacaggtgtgcaccaccatgcccagctaactcttgtatttttagtagagatggggtttctccatgttggccaggctggtctcagtgggccccagcgatccttccgcctcgggctcctgaatgactgggactacaggtgtgctactgcacctggctattttgaaataatttgacttagaagaatatttctacaattgtgttcaccttcttatgcaaatacaatcttcagtggcgctggcatatacaagctgagaaagtattgtcaagtgggttgtgccagcacatctgaccaggattttttgttgtagaaatattggatcctcacctgaggccaggagtttgagaccagcctggctaacatggtgaaactccgactctactaaaaatacaaaaattagctgggcgtggtggcaggtgcctgcagtcccagctgctcgggaggttgaggcaggagaatcgcttgaacccaggaggcggaggttgcggtgagccgagatcgcgccgctgcactctagcctgggcaatgaagtgagactctgtctcaaaaaacgaagtattagatcctcaatctcaaggtattctaagaaattttggagaccattgagtctaaaattcccagtatctttgaggcaggaacagacttggagaatgtagtttatgagcaggagtttggagctggaagaaatactgctttctgttggtggttaatgctgtcagctccttggattgtggctttagccctaaatattggggcagtagagactcttacctggaaaacaattgagggccacccatgttagcggcaagaggcagaggaaagcttggatggttgggctgaagatggtggatgtgctgtccctgtgagagtgctgatgctggactctggagccaacgacaaagtgtttgagcaagcagggtccaagcaagggcagtcgagggccggatgaagtgggcaggaaccgagtttcccaggtgacatcctgcctgtgctcatcacgccgaggggtgttgcacaatcacaccgattctttgtcactactgagtgcagtgttcttaagaatggggacctggcagctgggtgcgatggcttgtgcctgtaatcccaacactttgggaggctgaagtaggcagatcacgaggtcaggagtttgagaccagcctggccaacatagtgaaccctgtctctactaaaaatacaaaaaattagccaggcctggtggcaggcacctgtaattccagctactcgagaggctgaggcaggagaatcgcttgaaaccgggaggtggaggttgcagtgacccaagatcgtgccattgccccctggcctgggcgacagtgcgagactctcaaaaaaataagtaaataaataaaaggagacctaggcttgttgtgcttgttttttggttttgattttccagagtttgagggaaagttgacccatcctgtttattgtgcccttgaggaggaaacaaggcaaatccctactcttgtgggcaggggtgcgcaaacctgtcagtctgagatggctagaaccacatcctctataacttgagggggataatctatctatctatctatctatacctatatatatacacacacacacacagattaaaaaaaatatatatatatacagaggaatcctcccttacctatggtttcatcttacacagtttcagtacagtataataatctcctgtgcttaatttataaattgaactttataatttgtcaacatatggattctagctcagtaggtccaggtggggctcaagatacgcatttcaggccaggtgcggtggctcattcctgtaatcccagcactttgggaggccgaggtgggaggatcacttgagcccaggagttgagactaacctgggtaacagcaacattttgtctaccagaattttaaaaaattgggcgcggtggctcacacctgtaatcccagcacttcgggaggccaaggtgggcagcttggccaacatggtgaaagcccacctctactaaaagtacaaaatttaggcaggtgtggtggcatgcacctgtaatcccagctacttgggaggctgaggcaggagaattgcttgaacctgggaggtggaggttgcagtgagctgagatcatgcaactgcactcaagcctgggtgacagaatgagactccatctcaaaaaaaaaaaagtgtggtggcatgtacctgtggtcccagctggagaggttgaggctgcagtgagctgtgttcccaccactgcactccagcccgcaggcctgggaaacagaacaagactgtccccctgccctccccgcaaagcatttctgacaggctttctggtgataatgatgctgttggttcaacacctctcagagtaacgttctagagtttggcagagtcaaattatttctgaaggggaactttgtacaa

SEQ ID NO: 3 - protein, 526 aa, Homo sapiens
MASNDYTQQATQSYGAYPTQPGQGYSQQSSQPYGQQSYSGYSQSTDTSGYGQSSYSSYGQSQNTGYGTQSTPQGYGSTGGYGSSQSSQSSYGQQSSYPGYGQQPAPSSTSGSYGSSSQSSSYGQPQSGSYSQQPSYGGQQQSYGQQQSYNPPQGYGQQNQYNSSSGGGGGGGGGGNYGQDQSSMSSGGGSGGGYGNQDQSGGGGSGGYGQQDRGGRGRGGSGGGGGGGGGGYNRSSGGYEPRGRGGGRGGRGGMGGSDRGGFNKFGGPRDQGSRHDSEQDNSDNNTIFVQGLGENVTIESVADYFKQIGIIKTNKKTGQPMINLYTDRETGKLKGEATVSFDDPPSAKAAIDWFDGKEFSGNPIKVSFATRRADFNRGGGNGRGGRGRGGPMGRGGYGGGGSGGGGRGGFPSGGGGGGGQQRAGDWKCPNPTCENMNFSWRNECNQCKAPKPDGPGGGPGGSHMGGNYGDDRRGGRGGYDRGGYRGRGGDRGGFRGGRGGGDRGGFGPGKMDSRGEHRQDRRERPY

SEQ ID NO: 4-5 - skipped (2 entries)

SEQ ID NO: 6 - DNA, 17 bp, Artificial sequence
  Primer
tgcttgcttgcctgtgc

SEQ ID NO: 7 - DNA, 20 bp, Artificial sequence
  Primer
actgtaactctgctgtccgt

SEQ ID NO: 8 - DNA, 18 bp, Artificial sequence
  Probe
ttgaggccatgtccgcgc

SEQ ID NO: 9 - DNA, 20 bp, Artificial sequence
  Primer
ggcaaattcaacggcacagt

SEQ ID NO: 10 - DNA, 20 bp, Artificial sequence
  Primer
gggtctcgctcctggaagat

SEQ ID NO: 11 - DNA, 27 bp, Artificial sequence
  Probe
aaggccgagaatgggaagcttgtcatc

SEQ ID NO: 12 - DNA, 20 bp, Artificial sequence
  Synthetic oligonucleotide
gtttatctgaattcgccata

SEQ ID NO: 13 - DNA, 20 bp, Artificial sequence
  Synthetic oligonucleotide
gcaatgtcacctttcatacc

SEQ ID NO: 14 - DNA, 20 bp, Artificial sequence
  Synthetic oligonucleotide
agttccaacaccgctgagta

SEQ ID NO: 15 - DNA, 20 bp, Artificial sequence
  Synthetic oligonucleotide
gccatgtccgcgcacgcgcg

SEQ ID NO: 16 - DNA, 20 bp, Artificial sequence
  Synthetic oligonucleotide
ggactggctataaccactgt

SEQ ID NO: 17 - DNA, 20 bp, Artificial sequence
  Synthetic oligonucleotide
ctggccataagaagaatagc

SEQ ID NO: 18 - DNA, 20 bp, Artificial sequence
  Synthetic oligonucleotide
catagccgccagtcgagcca

SEQ ID NO: 19 - DNA, 20 bp, Artificial sequence
  Synthetic oligonucleotide
cccgtaagacgattgggagc

SEQ ID NO: 20 - DNA, 20 bp, Artificial sequence
  Synthetic oligonucleotide
tgagaactgctaccgtaact

SEQ ID NO: 21 - DNA, 20 bp, Artificial sequence
  Synthetic oligonucleotide
tgctgtccaccatagctagg

SEQ ID NO: 22 - DNA, 20 bp, Artificial sequence
  Synthetic oligonucleotide
caccactactcatggaggat

SEQ ID NO: 23 - DNA, 20 bp, Artificial sequence
  Synthetic oligonucleotide
ctgctgtccatagccaccgc

SEQ ID NO: 24 - DNA, 20 bp, Artificial sequence
  Synthetic oligonucleotide
gcggttgtaaccaccaccgc

SEQ ID NO: 25 - DNA, 20 bp, Artificial sequence
  Synthetic oligonucleotide
cgagtagcaaatgagacctt

SEQ ID NO: 26 - DNA, 20 bp, Artificial sequence
  Synthetic oligonucleotide
ccaccaccccgattaaagtc

SEQ ID NO: 27 - DNA, 20 bp, Artificial sequence
  Synthetic oligonucleotide
tgggaaatcctcctcggcca

SEQ ID NO: 28 - DNA, 20 bp, Artificial sequence
  Synthetic oligonucleotide
acgacgatcatccccgtagt

SEQ ID NO: 29 - DNA, 20 bp, Artificial sequence
  Synthetic oligonucleotide
ccgcctcgatcatagcctcc

SEQ ID NO: 30 - DNA, 20 bp, Artificial sequence
  Synthetic oligonucleotide
gccccggtagccgcctcgat

SEQ ID NO: 31 - DNA, 20 bp, Artificial sequence
  Synthetic oligonucleotide
ttaatacggcctctccctgc

SEQ ID NO: 32 - DNA, 20 bp, Artificial sequence
  Synthetic oligonucleotide
ccaggctaattaatacggcc

SEQ ID NO: 33 - DNA, 20 bp, Artificial sequence
  Synthetic oligonucleotide
tagtccgacacaaaaaaacc

SEQ ID NO: 34 - DNA, 20 bp, Artificial sequence
  Synthetic oligonucleotide
ttacaattacatagtccgac

SEQ ID NO: 35 - DNA, 20 bp, Artificial sequence
  Synthetic oligonucleotide
ggaaccagaggtatagttac

SEQ ID NO: 36 - DNA, 20 bp, Artificial sequence
  Synthetic oligonucleotide
tcgggacatcgatcttccag

SEQ ID NO: 37 - DNA, 20 bp, Artificial sequence
  Synthetic oligonucleotide
gcagggtaatctgaacagga

SEQ ID NO: 38 - DNA, 20 bp, Artificial sequence
  Synthetic oligonucleotide
atttggccttctccccgaac

SEQ ID NO: 39 - DNA, 20 bp, Artificial sequence
  Synthetic oligonucleotide
taggccaacactcatgacat

SEQ ID NO: 40 - DNA, 20 bp, Artificial sequence
  Synthetic oligonucleotide
gagtcactcacctcctagat

SEQ ID NO: 41 - DNA, 20 bp, Artificial sequence
  Synthetic oligonucleotide
gtcaatgacctcaagccctc

SEQ ID NO: 42 - DNA, 20 bp, Artificial sequence
  Synthetic oligonucleotide
cgtgcaagtttacaaccaca

SEQ ID NO: 43 - DNA, 20 bp, Artificial sequence
  Synthetic oligonucleotide
tcttacaaaccaagttcgaa

SEQ ID NO: 44 - DNA, 20 bp, Artificial sequence
  Synthetic oligonucleotide
ggaagtaaacctgctattcc

SEQ ID NO: 45 - DNA, 20 bp, Artificial sequence
  Synthetic oligonucleotide
accactctccgcctactgtt

SEQ ID NO: 46 - DNA, 20 bp, Artificial sequence
  Synthetic oligonucleotide
ttaatacgccagaccactct

SEQ ID NO: 47 - DNA, 20 bp, Artificial sequence
  Synthetic oligonucleotide
cccacttgacgatcctttgt

SEQ ID NO: 48 - DNA, 20 bp, Artificial sequence
  Synthetic oligonucleotide
agtgaactactcaaatatcg

SEQ ID NO: 49 - DNA, 20 bp, Artificial sequence
  Synthetic oligonucleotide
ggtcccagtaatcatatctt

SEQ ID NO: 50 - DNA, 20 bp, Artificial sequence
  Synthetic oligonucleotide
ggccaatcacatatgccatt

SEQ ID NO: 51 - DNA, 20 bp, Artificial sequence
  Synthetic oligonucleotide
actggacctacccactaaac

SEQ ID NO: 52 - DNA, 20 bp, Artificial sequence
  Synthetic oligonucleotide
tgggacacctaatgcttcaa

SEQ ID NO: 53 - DNA, 20 bp, Artificial sequence
  Synthetic oligonucleotide
gcagccctacatccaagtac

SEQ ID NO: 54 - DNA, 20 bp, Artificial sequence
  Synthetic oligonucleotide
ctggtcaatctacccaccac

SEQ ID NO: 55 - DNA, 20 bp, Artificial sequence
  Synthetic oligonucleotide
ccctagaccttaattcctgg

SEQ ID NO: 56 - DNA, 20 bp, Artificial sequence
  Synthetic oligonucleotide
attttcatagccggacacag

SEQ ID NO: 57 - DNA, 20 bp, Artificial sequence
  Synthetic oligonucleotide
tggccgggccccttcgctgg

SEQ ID NO: 58 - DNA, 20 bp, Artificial sequence
  Synthetic oligonucleotide
cgatctatctccacccccat

SEQ ID NO: 59 - DNA, 20 bp, Artificial sequence
  Synthetic oligonucleotide
gcaggactagcccacgatct

SEQ ID NO: 60 - DNA, 20 bp, Artificial sequence
  Synthetic oligonucleotide
gtcgaagcttaagtacgctc

SEQ ID NO: 61 - DNA, 20 bp, Artificial sequence
  Synthetic oligonucleotide
ctcgcgcccttacctaccgt

SEQ ID NO: 62 - DNA, 20 bp, Artificial sequence
  Synthetic oligonucleotide
cccggtcccactgaaaacga

SEQ ID NO: 63 - DNA, 20 bp, Artificial sequence
  Synthetic oligonucleotide
agacttcccgccccgcgcgc

SEQ ID NO: 64 - DNA, 20 bp, Artificial sequence
  Synthetic oligonucleotide
ggagcgatcccgcccattcg

SEQ ID NO: 65 - DNA, 20 bp, Artificial sequence
  Synthetic oligonucleotide
ccaccgccgccaaaccgtta

SEQ ID NO: 66 - DNA, 20 bp, Artificial sequence
  Synthetic oligonucleotide
gggccgtccccaagtccgtt

SEQ ID NO: 67 - DNA, 20 bp, Artificial sequence
  Synthetic oligonucleotide
cggccgttcttctccgtccc

SEQ ID NO: 68 - DNA, 20 bp, Artificial sequence
  Synthetic oligonucleotide
ggctttttagtgcaaagcca

SEQ ID NO: 69 - DNA, 20 bp, Artificial sequence
  Synthetic oligonucleotide
gtgattgctctaaaacatcg

SEQ ID NO: 70 - DNA, 20 bp, Artificial sequence
  Synthetic oligonucleotide
agttccaatttcaccccgcc

SEQ ID NO: 71 - DNA, 20 bp, Artificial sequence
  Synthetic oligonucleotide
ccgtaccttcccgaggtgct

SEQ ID NO: 72 - DNA, 20 bp, Artificial sequence
  Synthetic oligonucleotide
atcaacaccaccgtaccttc

SEQ ID NO: 73 - DNA, 20 bp, Artificial sequence
  Synthetic oligonucleotide
ggccatagttacctgtgaga

SEQ ID NO: 74 - DNA, 20 bp, Artificial sequence
  Synthetic oligonucleotide
atcatcggtttcccttgcag

SEQ ID NO: 75 - DNA, 20 bp, Artificial sequence
  Synthetic oligonucleotide
gcttacttcagtcagctggc

SEQ ID NO: 76 - DNA, 20 bp, Artificial sequence
  Synthetic oligonucleotide
gtcaccccttctacactgcg

SEQ ID NO: 77 - DNA, 20 bp, Artificial sequence
  Synthetic oligonucleotide
gttggtttaaaaaccctacc

SEQ ID NO: 78 - DNA, 20 bp, Artificial sequence
  Synthetic oligonucleotide
tacctgctccaggttagcac

SEQ ID NO: 79 - DNA, 20 bp, Artificial sequence
  Synthetic oligonucleotide
tccaaggcctactagacccc

SEQ ID NO: 80 - DNA, 20 bp, Artificial sequence
  Synthetic oligonucleotide
tcattgacaccattccgtac

SEQ ID NO: 81 - DNA, 20 bp, Artificial sequence
  Synthetic oligonucleotide
ggtccacgaattcagtttgt

SEQ ID NO: 82 - DNA, 20 bp, Artificial sequence
  Synthetic oligonucleotide
gttgtttccccgaaaccaca

SEQ ID NO: 83 - DNA, 20 bp, Artificial sequence
  Synthetic oligonucleotide
tgggctcgccaccagccatg

SEQ ID NO: 84 - DNA, 20 bp, Artificial sequence
  Synthetic oligonucleotide
ccaaaccctttcctgggtcg

SEQ ID NO: 85 - DNA, 20 bp, Artificial sequence
  Synthetic oligonucleotide
gggtcctctcagacctaaat

SEQ ID NO: 86 - DNA, 20 bp, Artificial sequence
  Synthetic oligonucleotide
ggtactctgataagttatac

SEQ ID NO: 87 - DNA, 20 bp, Artificial sequence
  Synthetic oligonucleotide
ggcttgtttcctaaggcttg

SEQ ID NO: 88 - DNA, 20 bp, Artificial sequence
  Synthetic oligonucleotide
cgcacatacctcagtaccaa

SEQ ID NO: 89 - DNA, 20 bp, Artificial sequence
  Synthetic oligonucleotide
gttccccgagcctccccgct

SEQ ID NO: 90 - DNA, 20 bp, Artificial sequence
  Synthetic oligonucleotide
accctgttatcctatggcct

SEQ ID NO: 91 - DNA, 20 bp, Artificial sequence
  Synthetic oligonucleotide
ccctcctacctaacccagcg

SEQ ID NO: 92 - DNA, 20 bp, Artificial sequence
  Synthetic oligonucleotide
cgaagttccaacaccgctga

SEQ ID NO: 93 - DNA, 20 bp, Artificial sequence
  Synthetic oligonucleotide
gtttgaggccatgtccgcgc

SEQ ID NO: 94 - DNA, 20 bp, Artificial sequence
  Synthetic oligonucleotide
gcctgaagtgtccgtggact

SEQ ID NO: 95 - DNA, 20 bp, Artificial sequence
  Synthetic oligonucleotide
cagtcgagccatatccctgg

SEQ ID NO: 96 - DNA, 20 bp, Artificial sequence
  Synthetic oligonucleotide
tgccatagccgccagtcgag

SEQ ID NO: 97 - DNA, 20 bp, Artificial sequence
  Synthetic oligonucleotide
gcccgtaagacgattgggag

SEQ ID NO: 98 - DNA, 20 bp, Artificial sequence
  Synthetic oligonucleotide
atagctaggctgctggctgt

SEQ ID NO: 99 - DNA, 20 bp, Artificial sequence
  Synthetic oligonucleotide
ctgctgtccaccatagctag

SEQ ID NO: 100 - DNA, 20 bp, Artificial sequence
  Synthetic oligonucleotide
cttgattgccataaccgcca

SEQ ID NO: 101 - DNA, 20 bp, Artificial sequence
  Synthetic oligonucleotide
cctgctgtccatagccaccg

SEQ ID NO: 102 - DNA, 20 bp, Artificial sequence
  Synthetic oligonucleotide
tgcggttgtaaccaccaccg

SEQ ID NO: 103 - DNA, 20 bp, Artificial sequence
  Synthetic oligonucleotide
gcgagtagcaaatgagacct

SEQ ID NO: 104 - DNA, 20 bp, Artificial sequence
  Synthetic oligonucleotide
gccaccaccccgattaaagt

SEQ ID NO: 105 - DNA, 20 bp, Artificial sequence
  Synthetic oligonucleotide
actgggaaatcctcctcggc

SEQ ID NO: 106 - DNA, 20 bp, Artificial sequence
  Synthetic oligonucleotide
cacgacgatcatccccgtag

SEQ ID NO: 107 - DNA, 20 bp, Artificial sequence
  Synthetic oligonucleotide
gccgcctcgatcatagcctc

SEQ ID NO: 108 - DNA, 20 bp, Artificial sequence
  Synthetic oligonucleotide
aagcctccacggtccccgcc

SEQ ID NO: 109 - DNA, 20 bp, Artificial sequence
  Synthetic oligonucleotide
attaatacggcctctccctg

SEQ ID NO: 110 - DNA, 20 bp, Artificial sequence
  Synthetic oligonucleotide
gccaggctaattaatacggc

SEQ ID NO: 111 - DNA, 20 bp, Artificial sequence
  Synthetic oligonucleotide
ttacatagtccgacacaaaa

SEQ ID NO: 112 - DNA, 20 bp, Artificial sequence
  Synthetic oligonucleotide
ggtcacttttaatgggaacc

SEQ ID NO: 113 - DNA, 20 bp, Artificial sequence
  Synthetic oligonucleotide
gatcgggacatcgatcttcc

SEQ ID NO: 114 - DNA, 20 bp, Artificial sequence
  Synthetic oligonucleotide
ccttctccccgaacactgta

SEQ ID NO: 115 - DNA, 20 bp, Artificial sequence
  Synthetic oligonucleotide
catttggccttctccccgaa

SEQ ID NO: 116 - DNA, 20 bp, Artificial sequence
  Synthetic oligonucleotide
ttaggccaacactcatgaca

SEQ ID NO: 117 - DNA, 20 bp, Artificial sequence
  Synthetic oligonucleotide
ggagtcactcacctcctaga

SEQ ID NO: 118 - DNA, 20 bp, Artificial sequence
  Synthetic oligonucleotide
cctccaatcaaaaagggatc

SEQ ID NO: 119 - DNA, 20 bp, Artificial sequence
  Synthetic oligonucleotide
gttacgctctgtgtaactaa

SEQ ID NO: 120 - DNA, 20 bp, Artificial sequence
  Synthetic oligonucleotide
gtcttacaaaccaagttcga

SEQ ID NO: 121 - DNA, 20 bp, Artificial sequence
  Synthetic oligonucleotide
gagagcaccccaatgctggc

SEQ ID NO: 122 - DNA, 20 bp, Artificial sequence
  Synthetic oligonucleotide
gaccactctccgcctactgt

SEQ ID NO: 123 - DNA, 20 bp, Artificial sequence
  Synthetic oligonucleotide
ttttaatacgccagaccact

SEQ ID NO: 124 - DNA, 20 bp, Artificial sequence
  Synthetic oligonucleotide
gcccacttgacgatcctttg

SEQ ID NO: 125 - DNA, 20 bp, Artificial sequence
  Synthetic oligonucleotide
gcaccaacagtgaactactc

SEQ ID NO: 126 - DNA, 20 bp, Artificial sequence
  Synthetic oligonucleotide
atggtcccagtaatcatatc

SEQ ID NO: 127 - DNA, 20 bp, Artificial sequence
  Synthetic oligonucleotide
gtcaaggccaatcacatatg

SEQ ID NO: 128 - DNA, 20 bp, Artificial sequence
  Synthetic oligonucleotide
aactggacctacccactaaa

SEQ ID NO: 129 - DNA, 20 bp, Artificial sequence
  Synthetic oligonucleotide
atgggacacctaatgcttca

SEQ ID NO: 130 - DNA, 20 bp, Artificial sequence
  Synthetic oligonucleotide
tgcagccctacatccaagta

SEQ ID NO: 131 - DNA, 20 bp, Artificial sequence
  Synthetic oligonucleotide
accttaattcctggtcaatc

SEQ ID NO: 132 - DNA, 20 bp, Artificial sequence
  Synthetic oligonucleotide
gaccctagaccttaattcct

SEQ ID NO: 133 - DNA, 20 bp, Artificial sequence
  Synthetic oligonucleotide
cccggatcctcatggctttg

SEQ ID NO: 134 - DNA, 20 bp, Artificial sequence
  Synthetic oligonucleotide
gtggccgggccccttcgctg

SEQ ID NO: 135 - DNA, 20 bp, Artificial sequence
  Synthetic oligonucleotide
gcccacgatctatctccacc

SEQ ID NO: 136 - DNA, 20 bp, Artificial sequence
  Synthetic oligonucleotide
ggaacgcactccgccccctt

SEQ ID NO: 137 - DNA, 20 bp, Artificial sequence
  Synthetic oligonucleotide
gcccttacctaccgtttgag

SEQ ID NO: 138 - DNA, 20 bp, Artificial sequence
  Synthetic oligonucleotide
cctcgcgcccttacctaccg

SEQ ID NO: 139 - DNA, 20 bp, Artificial sequence
  Synthetic oligonucleotide
cacgggatcgccgccccggt

SEQ ID NO: 140 - DNA, 20 bp, Artificial sequence
  Synthetic oligonucleotide
ctcgcgacagaaagctgaac

SEQ ID NO: 141 - DNA, 20 bp, Artificial sequence
  Synthetic oligonucleotide
cggagcgatcccgcccattc

SEQ ID NO: 142 - DNA, 20 bp, Artificial sequence
  Synthetic oligonucleotide
accaccgccgccaaaccgtt

SEQ ID NO: 143 - DNA, 20 bp, Artificial sequence
  Synthetic oligonucleotide
tcgggccgtccccaagtccg

SEQ ID NO: 144 - DNA, 20 bp, Artificial sequence
  Synthetic oligonucleotide
gcggccgttcttctccgtcc

SEQ ID NO: 145 - DNA, 20 bp, Artificial sequence
  Synthetic oligonucleotide
actctttgaccaatcccgga

SEQ ID NO: 146 - DNA, 20 bp, Artificial sequence
  Synthetic oligonucleotide
ggtggacatccacaattttc

SEQ ID NO: 147 - DNA, 20 bp, Artificial sequence
  Synthetic oligonucleotide
cagttccaatttcaccccgc

SEQ ID NO: 148 - DNA, 20 bp, Artificial sequence
  Synthetic oligonucleotide
accgtaccttcccgaggtgc

SEQ ID NO: 149 - DNA, 20 bp, Artificial sequence
  Synthetic oligonucleotide
ccgacatcaacaccaccgta

SEQ ID NO: 150 - DNA, 20 bp, Artificial sequence
  Synthetic oligonucleotide
ttggccatagttacctgtga

SEQ ID NO: 151 - DNA, 20 bp, Artificial sequence
  Synthetic oligonucleotide
tcaggttaaccattaccaac

SEQ ID NO: 152 - DNA, 20 bp, Artificial sequence
  Synthetic oligonucleotide
gtagggtccttcaaatctta

SEQ ID NO: 153 - DNA, 20 bp, Artificial sequence
  Synthetic oligonucleotide
ggtcaccccttctacactgc

SEQ ID NO: 154 - DNA, 20 bp, Artificial sequence
  Synthetic oligonucleotide
ggttgacaaccaagtagttg

SEQ ID NO: 155 - DNA, 20 bp, Artificial sequence
  Synthetic oligonucleotide
attgagtcttacccctacct

SEQ ID NO: 156 - DNA, 20 bp, Artificial sequence
  Synthetic oligonucleotide
gtccaaggcctactagaccc

SEQ ID NO: 157 - DNA, 20 bp, Artificial sequence
  Synthetic oligonucleotide
ttcattgacaccattccgta

SEQ ID NO: 158 - DNA, 20 bp, Artificial sequence
  Synthetic oligonucleotide
cacctaagtcatgaacccac

SEQ ID NO: 159 - DNA, 20 bp, Artificial sequence
  Synthetic oligonucleotide
ccgtgttgtttccccgaaac

SEQ ID NO: 160 - DNA, 20 bp, Artificial sequence
  Synthetic oligonucleotide
agatgggctcgccaccagcc

SEQ ID NO: 161 - DNA, 20 bp, Artificial sequence
  Synthetic oligonucleotide
gggcctttagtgacatggaa

SEQ ID NO: 162 - DNA, 20 bp, Artificial sequence
  Synthetic oligonucleotide
ggtccccgaattaaataaga

SEQ ID NO: 163 - DNA, 20 bp, Artificial sequence
  Synthetic oligonucleotide
gctacagtactccctttcca

SEQ ID NO: 164 - DNA, 20 bp, Artificial sequence
  Synthetic oligonucleotide
gcaagacacattaatccgaa

SEQ ID NO: 165 - DNA, 20 bp, Artificial sequence
  Synthetic oligonucleotide
acgcacatacctcagtacca

SEQ ID NO: 166 - DNA, 20 bp, Artificial sequence
  Synthetic oligonucleotide
ccattcccctatgttccccg

SEQ ID NO: 167 - DNA, 20 bp, Artificial sequence
  Synthetic oligonucleotide
aaccctgttatcctatggcc

SEQ ID NO: 168 - DNA, 20 bp, Artificial sequence
  Synthetic oligonucleotide
ctagatatcctatctgcccc

SEQ ID NO: 169 - DNA, 20 bp, Artificial sequence
  Synthetic oligonucleotide
acgaagttccaacaccgctg

SEQ ID NO: 170 - DNA, 20 bp, Artificial sequence
  Synthetic oligonucleotide
ctgggaatagccctgcccgg

SEQ ID NO: 171 - DNA, 20 bp, Artificial sequence
  Synthetic oligonucleotide
atagcctgaagtgtccgtgg

SEQ ID NO: 172 - DNA, 20 bp, Artificial sequence
  Synthetic oligonucleotide
ccagtcgagccatatccctg

SEQ ID NO: 173 - DNA, 20 bp, Artificial sequence
  Synthetic oligonucleotide
actgccatagccgccagtcg

SEQ ID NO: 174 - DNA, 20 bp, Artificial sequence
  Synthetic oligonucleotide
tgcccgtaagacgattggga

SEQ ID NO: 175 - DNA, 20 bp, Artificial sequence
  Synthetic oligonucleotide
ccatagctaggctgctggct

SEQ ID NO: 176 - DNA, 20 bp, Artificial sequence
  Synthetic oligonucleotide
gctgctgtccaccatagcta

SEQ ID NO: 177 - DNA, 20 bp, Artificial sequence
  Synthetic oligonucleotide
tcttgattgccataaccgcc

SEQ ID NO: 178 - DNA, 20 bp, Artificial sequence
  Synthetic oligonucleotide
cggtcctgctgtccatagcc

SEQ ID NO: 179 - DNA, 20 bp, Artificial sequence
  Synthetic oligonucleotide
gccacagactcaattgtaac

SEQ ID NO: 180 - DNA, 20 bp, Artificial sequence
  Synthetic oligonucleotide
gattaaagtctgcccggcga

SEQ ID NO: 181 - DNA, 20 bp, Artificial sequence
  Synthetic oligonucleotide
tgccaccaccccgattaaag

SEQ ID NO: 182 - DNA, 20 bp, Artificial sequence
  Synthetic oligonucleotide
cactgggaaatcctcctcgg

SEQ ID NO: 183 - DNA, 20 bp, Artificial sequence
  Synthetic oligonucleotide
ccacgacgatcatccccgta

SEQ ID NO: 184 - DNA, 20 bp, Artificial sequence
  Synthetic oligonucleotide
agccgcctcgatcatagcct

SEQ ID NO: 185 - DNA, 20 bp, Artificial sequence
  Synthetic oligonucleotide
ctcggaagcctccacggtcc

SEQ ID NO: 186 - DNA, 20 bp, Artificial sequence
  Synthetic oligonucleotide
taattaatacggcctctccc

SEQ ID NO: 187 - DNA, 20 bp, Artificial sequence
  Synthetic oligonucleotide
agccaggctaattaatacgg

SEQ ID NO: 188 - DNA, 20 bp, Artificial sequence
  Synthetic oligonucleotide
aattacatagtccgacacaa

SEQ ID NO: 189 - DNA, 20 bp, Artificial sequence
  Synthetic oligonucleotide
atcgatcttccaggaaagtg

SEQ ID NO: 190 - DNA, 20 bp, Artificial sequence
  Synthetic oligonucleotide
tctaccttcctgatcgggac

SEQ ID NO: 191 - DNA, 20 bp, Artificial sequence
  Synthetic oligonucleotide
gccttctccccgaacactgt

SEQ ID NO: 192 - DNA, 20 bp, Artificial sequence
  Synthetic oligonucleotide
tcatttggccttctccccga

SEQ ID NO: 193 - DNA, 20 bp, Artificial sequence
  Synthetic oligonucleotide
gcctcaccattaaaagggcc

SEQ ID NO: 194 - DNA, 20 bp, Artificial sequence
  Synthetic oligonucleotide
gggagtcactcacctcctag

SEQ ID NO: 195 - DNA, 20 bp, Artificial sequence
  Synthetic oligonucleotide
taggagggccttccaccctc

SEQ ID NO: 196 - DNA, 20 bp, Artificial sequence
  Synthetic oligonucleotide
ttaatgttacgctctgtgta

SEQ ID NO: 197 - DNA, 20 bp, Artificial sequence
  Synthetic oligonucleotide
tgtcttacaaaccaagttcg

SEQ ID NO: 198 - DNA, 20 bp, Artificial sequence
  Synthetic oligonucleotide
tctccgcctactgttgctta

SEQ ID NO: 199 - DNA, 20 bp, Artificial sequence
  Synthetic oligonucleotide
cgccagaccactctccgcct

SEQ ID NO: 200 - DNA, 20 bp, Artificial sequence
  Synthetic oligonucleotide
tttttaatacgccagaccac

SEQ ID NO: 201 - DNA, 20 bp, Artificial sequence
  Synthetic oligonucleotide
aaggcccacttgacgatcct

SEQ ID NO: 202 - DNA, 20 bp, Artificial sequence
  Synthetic oligonucleotide
gattagaatcctgctaggca

SEQ ID NO: 203 - DNA, 20 bp, Artificial sequence
  Synthetic oligonucleotide
acttgacactaatggtccca

SEQ ID NO: 204 - DNA, 20 bp, Artificial sequence
  Synthetic oligonucleotide
gacctacccactaaacagtc

SEQ ID NO: 205 - DNA, 20 bp, Artificial sequence
  Synthetic oligonucleotide
caaactggacctacccacta

SEQ ID NO: 206 - DNA, 20 bp, Artificial sequence
  Synthetic oligonucleotide
cttagcctgtcccaattcca

SEQ ID NO: 207 - DNA, 20 bp, Artificial sequence
  Synthetic oligonucleotide
ctgcagccctacatccaagt

SEQ ID NO: 208 - DNA, 20 bp, Artificial sequence
  Synthetic oligonucleotide
gaccttaattcctggtcaat

SEQ ID NO: 209 - DNA, 20 bp, Artificial sequence
  Synthetic oligonucleotide
ggaccctagaccttaattcc

SEQ ID NO: 210 - DNA, 20 bp, Artificial sequence
  Synthetic oligonucleotide
acccggatcctcatggcttt

SEQ ID NO: 211 - DNA, 20 bp, Artificial sequence
  Synthetic oligonucleotide
accgagattcctgtggccgg

SEQ ID NO: 212 - DNA, 20 bp, Artificial sequence
  Synthetic oligonucleotide
agcccacgatctatctccac

SEQ ID NO: 213 - DNA, 20 bp, Artificial sequence
  Synthetic oligonucleotide
ctccgccgcctacgcaccgc

SEQ ID NO: 214 - DNA, 20 bp, Artificial sequence
  Synthetic oligonucleotide
cgcccttacctaccgtttga

SEQ ID NO: 215 - DNA, 20 bp, Artificial sequence
  Synthetic oligonucleotide
gcctcgcgcccttacctacc

SEQ ID NO: 216 - DNA, 20 bp, Artificial sequence
  Synthetic oligonucleotide
cgcggcttcccgccacaggg

SEQ ID NO: 217 - DNA, 20 bp, Artificial sequence
  Synthetic oligonucleotide
cacaccggacgcgcgccgcc

SEQ ID NO: 218 - DNA, 20 bp, Artificial sequence
  Synthetic oligonucleotide
ggaacggagcgatcccgccc

SEQ ID NO: 219 - DNA, 20 bp, Artificial sequence
  Synthetic oligonucleotide
cgaaccctgaccaccgccgc

SEQ ID NO: 220 - DNA, 20 bp, Artificial sequence
  Synthetic oligonucleotide
actctcgggccgtccccaag

SEQ ID NO: 221 - DNA, 20 bp, Artificial sequence
  Synthetic oligonucleotide
agccccacttaagatacacg

SEQ ID NO: 222 - DNA, 20 bp, Artificial sequence
  Synthetic oligonucleotide
caggtttgaattcgaacagt

SEQ ID NO: 223 - DNA, 20 bp, Artificial sequence
  Synthetic oligonucleotide
cgttatcagccaagtgttct

SEQ ID NO: 224 - DNA, 20 bp, Artificial sequence
  Synthetic oligonucleotide
ctaccaactctttagtacag

SEQ ID NO: 225 - DNA, 20 bp, Artificial sequence
  Synthetic oligonucleotide
caccgtaccttcccgaggtg

SEQ ID NO: 226 - DNA, 20 bp, Artificial sequence
  Synthetic oligonucleotide
cccgacatcaacaccaccgt

SEQ ID NO: 227 - DNA, 20 bp, Artificial sequence
  Synthetic oligonucleotide
ggctcatgagacacctaccc

SEQ ID NO: 228 - DNA, 20 bp, Artificial sequence
  Synthetic oligonucleotide
gtcaggttaaccattaccaa

SEQ ID NO: 229 - DNA, 20 bp, Artificial sequence
  Synthetic oligonucleotide
cttaccatttccaaactcgg

SEQ ID NO: 230 - DNA, 20 bp, Artificial sequence
  Synthetic oligonucleotide
gggtcaccccttctacactg

SEQ ID NO: 231 - DNA, 20 bp, Artificial sequence
  Synthetic oligonucleotide
taccctacccctttctggag

SEQ ID NO: 232 - DNA, 20 bp, Artificial sequence
  Synthetic oligonucleotide
acccctcttattaacctggg

SEQ ID NO: 233 - DNA, 20 bp, Artificial sequence
  Synthetic oligonucleotide
gcaacggcccagtccaaggc

SEQ ID NO: 234 - DNA, 20 bp, Artificial sequence
  Synthetic oligonucleotide
gagctagtttctatttgccc

SEQ ID NO: 235 - DNA, 20 bp, Artificial sequence
  Synthetic oligonucleotide
gacacctaagtcatgaaccc

SEQ ID NO: 236 - DNA, 20 bp, Artificial sequence
  Synthetic oligonucleotide
accatccttaaaaccgtgtt

SEQ ID NO: 237 - DNA, 20 bp, Artificial sequence
  Synthetic oligonucleotide
cccggttctctcacccgaga

SEQ ID NO: 238 - DNA, 20 bp, Artificial sequence
  Synthetic oligonucleotide
cccgagggcctttagtgaca

SEQ ID NO: 239 - DNA, 20 bp, Artificial sequence
  Synthetic oligonucleotide
cctagtatccatcaagcaac

SEQ ID NO: 240 - DNA, 20 bp, Artificial sequence
  Synthetic oligonucleotide
gccttctcatacataccatc

SEQ ID NO: 241 - DNA, 20 bp, Artificial sequence
  Synthetic oligonucleotide
tgcaagacacattaatccga

SEQ ID NO: 242 - DNA, 20 bp, Artificial sequence
  Synthetic oligonucleotide
acatcaaccttacctaggta

SEQ ID NO: 243 - DNA, 20 bp, Artificial sequence
  Synthetic oligonucleotide
cccgtagttaccccctagga

SEQ ID NO: 244 - DNA, 20 bp, Artificial sequence
  Synthetic oligonucleotide
gcgagtatcttatctcaagt

SEQ ID NO: 245 - DNA, 20 bp, Artificial sequence
  Synthetic oligonucleotide
cctagatatcctatctgccc

SEQ ID NO: 246 - DNA, 20 bp, Artificial sequence
  Synthetic oligonucleotide
aacgaagttccaacaccgct

SEQ ID NO: 247 - DNA, 20 bp, Artificial sequence
  Synthetic oligonucleotide
actctgctgtccgtagggct

SEQ ID NO: 248 - DNA, 20 bp, Artificial sequence
  Synthetic oligonucleotide
ggccatagcctgaagtgtcc

SEQ ID NO: 249 - DNA, 20 bp, Artificial sequence
  Synthetic oligonucleotide
gccagtcgagccatatccct

SEQ ID NO: 250 - DNA, 20 bp, Artificial sequence
  Synthetic oligonucleotide
ggctactgccatagccgcca

SEQ ID NO: 251 - DNA, 20 bp, Artificial sequence
  Synthetic oligonucleotide
gactgctgcccgtaagacga

SEQ ID NO: 252 - DNA, 20 bp, Artificial sequence
  Synthetic oligonucleotide
accatagctaggctgctggc

SEQ ID NO: 253 - DNA, 20 bp, Artificial sequence
  Synthetic oligonucleotide
gatcttggccatagttacct

SEQ ID NO: 254 - DNA, 20 bp, Artificial sequence
  Synthetic oligonucleotide
gtcttgattgccataaccgc

SEQ ID NO: 255 - DNA, 20 bp, Artificial sequence
  Synthetic oligonucleotide
ccacggtcctgctgtccata

SEQ ID NO: 256 - DNA, 20 bp, Artificial sequence
  Synthetic oligonucleotide
ggctgtcccgttttcttgtt

SEQ ID NO: 257 - DNA, 20 bp, Artificial sequence
  Synthetic oligonucleotide
caccccgattaaagtctgcc

SEQ ID NO: 258 - DNA, 20 bp, Artificial sequence
  Synthetic oligonucleotide
cggcctccacgaccattgcc

SEQ ID NO: 259 - DNA, 20 bp, Artificial sequence
  Synthetic oligonucleotide
gattaggacacttccagtca

SEQ ID NO: 260 - DNA, 20 bp, Artificial sequence
  Synthetic oligonucleotide
accacgacgatcatccccgt

SEQ ID NO: 261 - DNA, 20 bp, Artificial sequence
  Synthetic oligonucleotide
tagccgcctcgatcatagcc

SEQ ID NO: 262 - DNA, 20 bp, Artificial sequence
  Synthetic oligonucleotide
cctcggaagcctccacggtc

SEQ ID NO: 263 - DNA, 20 bp, Artificial sequence
  Synthetic oligonucleotide
ctaattaatacggcctctcc

SEQ ID NO: 264 - DNA, 20 bp, Artificial sequence
  Synthetic oligonucleotide
ggttacaaaataacgagggt

SEQ ID NO: 265 - DNA, 20 bp, Artificial sequence
  Synthetic oligonucleotide
caattacatagtccgacaca

SEQ ID NO: 266 - DNA, 20 bp, Artificial sequence
  Synthetic oligonucleotide
gacatcgatcttccaggaaa

SEQ ID NO: 267 - DNA, 20 bp, Artificial sequence
  Synthetic oligonucleotide
ctctaccttcctgatcggga

SEQ ID NO: 268 - DNA, 20 bp, Artificial sequence
  Synthetic oligonucleotide
ggccttctccccgaacactg

SEQ ID NO: 269 - DNA, 20 bp, Artificial sequence
  Synthetic oligonucleotide
ctcaaggatatcatttggcc

SEQ ID NO: 270 - DNA, 20 bp, Artificial sequence
  Synthetic oligonucleotide
cgctctccaccatggtcaaa

SEQ ID NO: 271 - DNA, 20 bp, Artificial sequence
  Synthetic oligonucleotide
cagaccagtctccttatagc

SEQ ID NO: 272 - DNA, 20 bp, Artificial sequence
  Synthetic oligonucleotide
ttaggagggccttccaccct

SEQ ID NO: 273 - DNA, 20 bp, Artificial sequence
  Synthetic oligonucleotide
ggttaatgttacgctctgtg

SEQ ID NO: 274 - DNA, 20 bp, Artificial sequence
  Synthetic oligonucleotide
gcaactcttcagtagagaac

SEQ ID NO: 275 - DNA, 20 bp, Artificial sequence
  Synthetic oligonucleotide
actctccgcctactgttgct

SEQ ID NO: 276 - DNA, 20 bp, Artificial sequence
  Synthetic oligonucleotide
acgccagaccactctccgcc

SEQ ID NO: 277 - DNA, 20 bp, Artificial sequence
  Synthetic oligonucleotide
gtttttaatacgccagacca

SEQ ID NO: 278 - DNA, 20 bp, Artificial sequence
  Synthetic oligonucleotide
gggaaggcccacttgacgat

SEQ ID NO: 279 - DNA, 20 bp, Artificial sequence
  Synthetic oligonucleotide
agattagaatcctgctaggc

SEQ ID NO: 280 - DNA, 20 bp, Artificial sequence
  Synthetic oligonucleotide
aacttgacactaatggtccc

SEQ ID NO: 281 - DNA, 20 bp, Artificial sequence
  Synthetic oligonucleotide
ggacctacccactaaacagt

SEQ ID NO: 282 - DNA, 20 bp, Artificial sequence
  Synthetic oligonucleotide
agatccccccaaactggacc

SEQ ID NO: 283 - DNA, 20 bp, Artificial sequence
  Synthetic oligonucleotide
cctacttagcctgtcccaat

SEQ ID NO: 284 - DNA, 20 bp, Artificial sequence
  Synthetic oligonucleotide
gtcaatctacccaccactga

SEQ ID NO: 285 - DNA, 20 bp, Artificial sequence
  Synthetic oligonucleotide
agaccttaattcctggtcaa

SEQ ID NO: 286 - DNA, 20 bp, Artificial sequence
  Synthetic oligonucleotide
gggctggaccctagacctta

SEQ ID NO: 287 - DNA, 20 bp, Artificial sequence
  Synthetic oligonucleotide
cacccggatcctcatggctt

SEQ ID NO: 288 - DNA, 20 bp, Artificial sequence
  Synthetic oligonucleotide
aaccgagattcctgtggccg

SEQ ID NO: 289 - DNA, 20 bp, Artificial sequence
  Synthetic oligonucleotide
tagcccacgatctatctcca

SEQ ID NO: 290 - DNA, 20 bp, Artificial sequence
  Synthetic oligonucleotide
gctccgccgcctacgcaccg

SEQ ID NO: 291 - DNA, 20 bp, Artificial sequence
  Synthetic oligonucleotide
gcgcccttacctaccgtttg

SEQ ID NO: 292 - DNA, 20 bp, Artificial sequence
  Synthetic oligonucleotide
tcgcctcgcgcccttaccta

SEQ ID NO: 293 - DNA, 20 bp, Artificial sequence
  Synthetic oligonucleotide
ccgcggcttcccgccacagg

SEQ ID NO: 294 - DNA, 20 bp, Artificial sequence
  Synthetic oligonucleotide
aaggctcacaccggacgcgc

SEQ ID NO: 295 - DNA, 20 bp, Artificial sequence
  Synthetic oligonucleotide
cgatcccgagcctccgcccc

SEQ ID NO: 296 - DNA, 20 bp, Artificial sequence
  Synthetic oligonucleotide
ggtcgaaccctgaccaccgc

SEQ ID NO: 297 - DNA, 20 bp, Artificial sequence
  Synthetic oligonucleotide
cgttcttctccgtccctatc

SEQ ID NO: 298 - DNA, 20 bp, Artificial sequence
  Synthetic oligonucleotide
tgggactccagatggttccg

SEQ ID NO: 299 - DNA, 20 bp, Artificial sequence
  Synthetic oligonucleotide
agccattatcgccaggagtc

SEQ ID NO: 300 - DNA, 20 bp, Artificial sequence
  Synthetic oligonucleotide
cgtgatcagaaaacatggcg

SEQ ID NO: 301 - DNA, 20 bp, Artificial sequence
  Synthetic oligonucleotide
gcaaagatagttaccctcct

SEQ ID NO: 302 - DNA, 20 bp, Artificial sequence
  Synthetic oligonucleotide
ccaccgtaccttcccgaggt

SEQ ID NO: 303 - DNA, 20 bp, Artificial sequence
  Synthetic oligonucleotide
gccttccccgacatcaacac

SEQ ID NO: 304 - DNA, 20 bp, Artificial sequence
  Synthetic oligonucleotide
gccctcacagatccctagac

SEQ ID NO: 305 - DNA, 20 bp, Artificial sequence
  Synthetic oligonucleotide
agtcaggttaaccattacca

SEQ ID NO: 306 - DNA, 20 bp, Artificial sequence
  Synthetic oligonucleotide
gtcacctttcatacctgtgg

SEQ ID NO: 307 - DNA, 20 bp, Artificial sequence
  Synthetic oligonucleotide
gtcctaactactgagctgtt

SEQ ID NO: 308 - DNA, 20 bp, Artificial sequence
  Synthetic oligonucleotide
ggcattctaccctacccctt

SEQ ID NO: 309 - DNA, 20 bp, Artificial sequence
  Synthetic oligonucleotide
gacccctcttattaacctgg

SEQ ID NO: 310 - DNA, 20 bp, Artificial sequence
  Synthetic oligonucleotide
tggcaacggcccagtccaag

SEQ ID NO: 311 - DNA, 20 bp, Artificial sequence
  Synthetic oligonucleotide
gacctggttatttcccatga

SEQ ID NO: 312 - DNA, 20 bp, Artificial sequence
  Synthetic oligonucleotide
gcaatgacacctaagtcatg

SEQ ID NO: 313 - DNA, 20 bp, Artificial sequence
  Synthetic oligonucleotide
aaccatccttaaaaccgtgt

SEQ ID NO: 314 - DNA, 20 bp, Artificial sequence
  Synthetic oligonucleotide
gcccggttctctcacccgag

SEQ ID NO: 315 - DNA, 20 bp, Artificial sequence
  Synthetic oligonucleotide
atccttggtcccgagggcct

SEQ ID NO: 316 - DNA, 20 bp, Artificial sequence
  Synthetic oligonucleotide
gcacctagtatccatcaagc

SEQ ID NO: 317 - DNA, 20 bp, Artificial sequence
  Synthetic oligonucleotide
gccagccttctcatacatac

SEQ ID NO: 318 - DNA, 20 bp, Artificial sequence
  Synthetic oligonucleotide
ttccggagaattctttacct

SEQ ID NO: 319 - DNA, 20 bp, Artificial sequence
  Synthetic oligonucleotide
tacatcaaccttacctaggt

SEQ ID NO: 320 - DNA, 20 bp, Artificial sequence
  Synthetic oligonucleotide
ccccgtagttaccccctagg

SEQ ID NO: 321 - DNA, 20 bp, Artificial sequence
  Synthetic oligonucleotide
agcgagtatcttatctcaag

SEQ ID NO: 322 - DNA, 20 bp, Artificial sequence
  Synthetic oligonucleotide
gcctagatatcctatctgcc

SEQ ID NO: 323 - DNA, 20 bp, Artificial sequence
  Synthetic oligonucleotide
caacgaagttccaacaccgc

SEQ ID NO: 324 - DNA, 20 bp, Artificial sequence
  Synthetic oligonucleotide
ggctataaccactgtaactc

SEQ ID NO: 325 - DNA, 20 bp, Artificial sequence
  Synthetic oligonucleotide
tggccatagcctgaagtgtc

SEQ ID NO: 326 - DNA, 20 bp, Artificial sequence
  Synthetic oligonucleotide
tagccgccagtcgagccata

SEQ ID NO: 327 - DNA, 20 bp, Artificial sequence
  Synthetic oligonucleotide
tggctactgccatagccgcc

SEQ ID NO: 328 - DNA, 20 bp, Artificial sequence
  Synthetic oligonucleotide
ggactgctgcccgtaagacg

SEQ ID NO: 329 - DNA, 20 bp, Artificial sequence
  Synthetic oligonucleotide
gtccaccatagctaggctgc

SEQ ID NO: 330 - DNA, 20 bp, Artificial sequence
  Synthetic oligonucleotide
catggaggattgatcttggc

SEQ ID NO: 331 - DNA, 20 bp, Artificial sequence
  Synthetic oligonucleotide
tggtcttgattgccataacc

SEQ ID NO: 332 - DNA, 20 bp, Artificial sequence
  Synthetic oligonucleotide
gccgcggcctccacggtcct

SEQ ID NO: 333 - DNA, 20 bp, Artificial sequence
  Synthetic oligonucleotide
gggctgtcccgttttcttgt

SEQ ID NO: 334 - DNA, 20 bp, Artificial sequence
  Synthetic oligonucleotide
accaccccgattaaagtctg

SEQ ID NO: 335 - DNA, 20 bp, Artificial sequence
  Synthetic oligonucleotide
tcggcctccacgaccattgc

SEQ ID NO: 336 - DNA, 20 bp, Artificial sequence
  Synthetic oligonucleotide
acgatcatccccgtagttac

SEQ ID NO: 337 - DNA, 20 bp, Artificial sequence
  Synthetic oligonucleotide
caccacgacgatcatccccg

SEQ ID NO: 338 - DNA, 20 bp, Artificial sequence
  Synthetic oligonucleotide
ggtagccgcctcgatcatag

SEQ ID NO: 339 - DNA, 20 bp, Artificial sequence
  Synthetic oligonucleotide
accaccccggccccctcgga

SEQ ID NO: 340 - DNA, 20 bp, Artificial sequence
  Synthetic oligonucleotide
ggctaattaatacggcctct

SEQ ID NO: 341 - DNA, 20 bp, Artificial sequence
  Synthetic oligonucleotide
aggttacaaaataacgaggg

SEQ ID NO: 342 - DNA, 20 bp, Artificial sequence
  Synthetic oligonucleotide
gttacaattacatagtccga

SEQ ID NO: 343 - DNA, 20 bp, Artificial sequence
  Synthetic oligonucleotide
gggacatcgatcttccagga

SEQ ID NO: 344 - DNA, 20 bp, Artificial sequence
  Synthetic oligonucleotide
tctctaccttcctgatcggg

SEQ ID NO: 345 - DNA, 20 bp, Artificial sequence
  Synthetic oligonucleotide
ttggccttctccccgaacac

SEQ ID NO: 346 - DNA, 20 bp, Artificial sequence
  Synthetic oligonucleotide
gccaacactcatgacatccc

SEQ ID NO: 347 - DNA, 20 bp, Artificial sequence
  Synthetic oligonucleotide
gcgctctccaccatggtcaa

SEQ ID NO: 348 - DNA, 20 bp, Artificial sequence
  Synthetic oligonucleotide
gccagaccagtctccttata

SEQ ID NO: 349 - DNA, 20 bp, Artificial sequence
  Synthetic oligonucleotide
ggttttaactcattggctgc

SEQ ID NO: 350 - DNA, 20 bp, Artificial sequence
  Synthetic oligonucleotide
tcttgggttaatgttacgct

SEQ ID NO: 351 - DNA, 20 bp, Artificial sequence
  Synthetic oligonucleotide
tcccagctatcgcttgaacc

SEQ ID NO: 352 - DNA, 20 bp, Artificial sequence
  Synthetic oligonucleotide
cactctccgcctactgttgc

SEQ ID NO: 353 - DNA, 20 bp, Artificial sequence
  Synthetic oligonucleotide
atacgccagaccactctccg

SEQ ID NO: 354 - DNA, 20 bp, Artificial sequence
  Synthetic oligonucleotide
tgtttttaatacgccagacc

SEQ ID NO: 355 - DNA, 20 bp, Artificial sequence
  Synthetic oligonucleotide
tgggaaggcccacttgacga

SEQ ID NO: 356 - DNA, 20 bp, Artificial sequence
  Synthetic oligonucleotide
cactcctaacaggagggcat

SEQ ID NO: 357 - DNA, 20 bp, Artificial sequence
  Synthetic oligonucleotide
gaacttgacactaatggtcc

SEQ ID NO: 358 - DNA, 20 bp, Artificial sequence
  Synthetic oligonucleotide
tggacctacccactaaacag

SEQ ID NO: 359 - DNA, 20 bp, Artificial sequence
  Synthetic oligonucleotide
gctaggtgtctctatccatt

SEQ ID NO: 360 - DNA, 20 bp, Artificial sequence
  Synthetic oligonucleotide
tcctacttagcctgtcccaa

SEQ ID NO: 361 - DNA, 20 bp, Artificial sequence
  Synthetic oligonucleotide
ggtcaatctacccaccactg

SEQ ID NO: 362 - DNA, 20 bp, Artificial sequence
  Synthetic oligonucleotide
tagaccttaattcctggtca

SEQ ID NO: 363 - DNA, 20 bp, Artificial sequence
  Synthetic oligonucleotide
gtcaagtctcacatgggctg

SEQ ID NO: 364 - DNA, 20 bp, Artificial sequence
  Synthetic oligonucleotide
tcacccggatcctcatggct

SEQ ID NO: 365 - DNA, 20 bp, Artificial sequence
  Synthetic oligonucleotide
ggaaccgagattcctgtggc

SEQ ID NO: 366 - DNA, 20 bp, Artificial sequence
  Synthetic oligonucleotide
actagcccacgatctatctc

SEQ ID NO: 367 - DNA, 20 bp, Artificial sequence
  Synthetic oligonucleotide
gtacgctccgccgcctacgc

SEQ ID NO: 368 - DNA, 20 bp, Artificial sequence
  Synthetic oligonucleotide
cgcgcccttacctaccgttt

SEQ ID NO: 369 - DNA, 20 bp, Artificial sequence
  Synthetic oligonucleotide
ccgtcgcctcgcgcccttac

SEQ ID NO: 370 - DNA, 20 bp, Artificial sequence
  Synthetic oligonucleotide
tccgcggcttcccgccacag

SEQ ID NO: 371 - DNA, 20 bp, Artificial sequence
  Synthetic oligonucleotide
ccgcccattcgcgaaggacc

SEQ ID NO: 372 - DNA, 20 bp, Artificial sequence
  Synthetic oligonucleotide
gagggcggccccgatcccga

SEQ ID NO: 373 - DNA, 20 bp, Artificial sequence
  Synthetic oligonucleotide
tggtcgaaccctgaccaccg

SEQ ID NO: 374 - DNA, 20 bp, Artificial sequence
  Synthetic oligonucleotide
ccgttcttctccgtccctat

SEQ ID NO: 375 - DNA, 20 bp, Artificial sequence
  Synthetic oligonucleotide
aactgctcgccttaggaggc

SEQ ID NO: 376 - DNA, 20 bp, Artificial sequence
  Synthetic oligonucleotide
gattgctctaaaacatcgcg

SEQ ID NO: 377 - DNA, 20 bp, Artificial sequence
  Synthetic oligonucleotide
cgtgcagtatctacaggaca

SEQ ID NO: 378 - DNA, 20 bp, Artificial sequence
  Synthetic oligonucleotide
gctgttagtgatgttgcaac

SEQ ID NO: 379 - DNA, 20 bp, Artificial sequence
  Synthetic oligonucleotide
accaccgtaccttcccgagg

SEQ ID NO: 380 - DNA, 20 bp, Artificial sequence
  Synthetic oligonucleotide
tcaagccttccccgacatca

SEQ ID NO: 381 - DNA, 20 bp, Artificial sequence
  Synthetic oligonucleotide
gcctaggatattaatgactc

SEQ ID NO: 382 - DNA, 20 bp, Artificial sequence
  Synthetic oligonucleotide
ggccccataaaccaagtcac

SEQ ID NO: 383 - DNA, 20 bp, Artificial sequence
  Synthetic oligonucleotide
cggagtattttgcaatgtca

SEQ ID NO: 384 - DNA, 20 bp, Artificial sequence
  Synthetic oligonucleotide
aggcaacttccccttaaagc

SEQ ID NO: 385 - DNA, 20 bp, Artificial sequence
  Synthetic oligonucleotide
aggtggcattctaccctacc

SEQ ID NO: 386 - DNA, 20 bp, Artificial sequence
  Synthetic oligonucleotide
tagacccctcttattaacct

SEQ ID NO: 387 - DNA, 20 bp, Artificial sequence
  Synthetic oligonucleotide
acaacgatcaaaaggatcct

SEQ ID NO: 388 - DNA, 20 bp, Artificial sequence
  Synthetic oligonucleotide
tccacgaattcagtttgtgc

SEQ ID NO: 389 - DNA, 20 bp, Artificial sequence
  Synthetic oligonucleotide
cgccaccagccatgcgatgt

SEQ ID NO: 390 - DNA, 20 bp, Artificial sequence
  Synthetic oligonucleotide
ggcccggttctctcacccga

SEQ ID NO: 391 - DNA, 20 bp, Artificial sequence
  Synthetic oligonucleotide
gtcttgataccactttagcc

SEQ ID NO: 392 - DNA, 20 bp, Artificial sequence
  Synthetic oligonucleotide
ggcaaccattaaagacttgc

SEQ ID NO: 393 - DNA, 20 bp, Artificial sequence
  Synthetic oligonucleotide
gcttgctgccctatatcccc

SEQ ID NO: 394 - DNA, 20 bp, Artificial sequence
  Synthetic oligonucleotide
ccatgcaagcctttaccatc

SEQ ID NO: 395 - DNA, 20 bp, Artificial sequence
  Synthetic oligonucleotide
cccattacatcaaccttacc

SEQ ID NO: 396 - DNA, 20 bp, Artificial sequence
  Synthetic oligonucleotide
atccccgtagttacccccta

SEQ ID NO: 397 - DNA, 20 bp, Artificial sequence
  Synthetic oligonucleotide
acctaacccagcgagtatct

SEQ ID NO: 398 - DNA, 20 bp, Artificial sequence
  Synthetic oligonucleotide
agcctagatatcctatctgc

SEQ ID NO: 399 - DNA, 20 bp, Artificial sequence
  Synthetic oligonucleotide
acgcgcgcacaggcaagcaa

SEQ ID NO: 400 - DNA, 20 bp, Artificial sequence
  Synthetic oligonucleotide
ctggctataaccactgtaac

SEQ ID NO: 401 - DNA, 20 bp, Artificial sequence
  Synthetic oligonucleotide
ctggccatagcctgaagtgt

SEQ ID NO: 402 - DNA, 20 bp, Artificial sequence
  Synthetic oligonucleotide
atagccgccagtcgagccat

SEQ ID NO: 403 - DNA, 20 bp, Artificial sequence
  Synthetic oligonucleotide
ctggctactgccatagccgc

SEQ ID NO: 404 - DNA, 20 bp, Artificial sequence
  Synthetic oligonucleotide
aggactgctgcccgtaagac

SEQ ID NO: 405 - DNA, 20 bp, Artificial sequence
  Synthetic oligonucleotide
gctgtccaccatagctaggc

SEQ ID NO: 406 - DNA, 20 bp, Artificial sequence
  Synthetic oligonucleotide
accactactcatggaggatt

SEQ ID NO: 407 - DNA, 20 bp, Artificial sequence
  Synthetic oligonucleotide
gctgtccatagccaccgctg

SEQ ID NO: 408 - DNA, 20 bp, Artificial sequence
  Synthetic oligonucleotide
tgccgcggcctccacggtcc

SEQ ID NO: 409 - DNA, 20 bp, Artificial sequence
  Synthetic oligonucleotide
aagagaccgttgcctctccc

SEQ ID NO: 410 - DNA, 20 bp, Artificial sequence
  Synthetic oligonucleotide
caccaccccgattaaagtct

SEQ ID NO: 411 - DNA, 20 bp, Artificial sequence
  Synthetic oligonucleotide
ctcggcctccacgaccattg

SEQ ID NO: 412 - DNA, 20 bp, Artificial sequence
  Synthetic oligonucleotide
gacgatcatccccgtagtta

SEQ ID NO: 413 - DNA, 20 bp, Artificial sequence
  Synthetic oligonucleotide
tcgatcatagcctcctctgc

SEQ ID NO: 414 - DNA, 20 bp, Artificial sequence
  Synthetic oligonucleotide
cggtagccgcctcgatcata

SEQ ID NO: 415 - DNA, 20 bp, Artificial sequence
  Synthetic oligonucleotide
atacggcctctccctgcgat

SEQ ID NO: 416 - DNA, 20 bp, Artificial sequence
  Synthetic oligonucleotide
caggctaattaatacggcct

SEQ ID NO: 417 - DNA, 20 bp, Artificial sequence
  Synthetic oligonucleotide
cccttgggtgatcaggaatt

SEQ ID NO: 418 - DNA, 20 bp, Artificial sequence
  Synthetic oligonucleotide
agttacaattacatagtccg

SEQ ID NO: 419 - DNA, 20 bp, Artificial sequence
  Synthetic oligonucleotide
cgggacatcgatcttccagg

SEQ ID NO: 420 - DNA, 20 bp, Artificial sequence
  Synthetic oligonucleotide
ctctctaccttcctgatcgg

SEQ ID NO: 421 - DNA, 20 bp, Artificial sequence
  Synthetic oligonucleotide
tttggccttctccccgaaca

SEQ ID NO: 422 - DNA, 20 bp, Artificial sequence
  Synthetic oligonucleotide
ggccaacactcatgacatcc

SEQ ID NO: 423 - DNA, 20 bp, Artificial sequence
  Synthetic oligonucleotide
actcacctcctagatcctga

SEQ ID NO: 424 - DNA, 20 bp, Artificial sequence
  Synthetic oligonucleotide
gtaacccagccagaccagtc

SEQ ID NO: 425 - DNA, 20 bp, Artificial sequence
  Synthetic oligonucleotide
aggttttaactcattggctg

SEQ ID NO: 426 - DNA, 20 bp, Artificial sequence
  Synthetic oligonucleotide
ctcttgggttaatgttacgc

SEQ ID NO: 427 - DNA, 20 bp, Artificial sequence
  Synthetic oligonucleotide
atcccagctatcgcttgaac

SEQ ID NO: 428 - DNA, 20 bp, Artificial sequence
  Synthetic oligonucleotide
ccactctccgcctactgttg

SEQ ID NO: 429 - DNA, 20 bp, Artificial sequence
  Synthetic oligonucleotide
aatacgccagaccactctcc

SEQ ID NO: 430 - DNA, 20 bp, Artificial sequence
  Synthetic oligonucleotide
cacttgacgatcctttgttt

SEQ ID NO: 431 - DNA, 20 bp, Artificial sequence
  Synthetic oligonucleotide
gtatcaggccatttcaacta

SEQ ID NO: 432 - DNA, 20 bp, Artificial sequence
  Synthetic oligonucleotide
caaggagcttcgacctcctc

SEQ ID NO: 433 - DNA, 20 bp, Artificial sequence
  Synthetic oligonucleotide
ggaacttgacactaatggtc

SEQ ID NO: 434 - DNA, 20 bp, Artificial sequence
  Synthetic oligonucleotide
ctggacctacccactaaaca

SEQ ID NO: 435 - DNA, 20 bp, Artificial sequence
  Synthetic oligonucleotide
ctgctaggtgtctctatcca

SEQ ID NO: 436 - DNA, 20 bp, Artificial sequence
  Synthetic oligonucleotide
gccctacatccaagtactga

SEQ ID NO: 437 - DNA, 20 bp, Artificial sequence
  Synthetic oligonucleotide
tggtcaatctacccaccact

SEQ ID NO: 438 - DNA, 20 bp, Artificial sequence
  Synthetic oligonucleotide
ctagaccttaattcctggtc

SEQ ID NO: 439 - DNA, 20 bp, Artificial sequence
  Synthetic oligonucleotide
gagtcaagtctcacatgggc

SEQ ID NO: 440 - DNA, 20 bp, Artificial sequence
  Synthetic oligonucleotide
gttgccttgcctttcggcct

SEQ ID NO: 441 - DNA, 20 bp, Artificial sequence
  Synthetic oligonucleotide
gtggtacggcctgagtgccc

SEQ ID NO: 442 - DNA, 20 bp, Artificial sequence
  Synthetic oligonucleotide
aggactagcccacgatctat

SEQ ID NO: 443 - DNA, 20 bp, Artificial sequence
  Synthetic oligonucleotide
gcttaagtacgctccgccgc

SEQ ID NO: 444 - DNA, 20 bp, Artificial sequence
  Synthetic oligonucleotide
tcgcgcccttacctaccgtt

SEQ ID NO: 445 - DNA, 20 bp, Artificial sequence
  Synthetic oligonucleotide
cgccgtcgcctcgcgccctt

SEQ ID NO: 446 - DNA, 20 bp, Artificial sequence
  Synthetic oligonucleotide
acttcccgccccgcgcgcga

SEQ ID NO: 447 - DNA, 20 bp, Artificial sequence
  Synthetic oligonucleotide
gcgatcccgcccattcgcga

SEQ ID NO: 448 - DNA, 20 bp, Artificial sequence
  Synthetic oligonucleotide
agagggcggccccgatcccg

SEQ ID NO: 449 - DNA, 20 bp, Artificial sequence
  Synthetic oligonucleotide
tccgttggtcgaaccctgac

SEQ ID NO: 450 - DNA, 20 bp, Artificial sequence
  Synthetic oligonucleotide
gccgttcttctccgtcccta

SEQ ID NO: 451 - DNA, 20 bp, Artificial sequence
  Synthetic oligonucleotide
gcaactgctcgccttaggag

SEQ ID NO: 452 - DNA, 20 bp, Artificial sequence
  Synthetic oligonucleotide
tgattgctctaaaacatcgc

SEQ ID NO: 453 - DNA, 20 bp, Artificial sequence
  Synthetic oligonucleotide
gttccaatttcaccccgcca

SEQ ID NO: 454 - DNA, 20 bp, Artificial sequence
  Synthetic oligonucleotide
gactgagttccatagcctgc

SEQ ID NO: 455 - DNA, 20 bp, Artificial sequence
  Synthetic oligonucleotide
caccaccgtaccttcccgag

SEQ ID NO: 456 - DNA, 20 bp, Artificial sequence
  Synthetic oligonucleotide
aggctcccctaccccaatta

SEQ ID NO: 457 - DNA, 20 bp, Artificial sequence
  Synthetic oligonucleotide
tcatcggtttcccttgcaga

SEQ ID NO: 458 - DNA, 20 bp, Artificial sequence
  Synthetic oligonucleotide
tcagctggccccataaacca

SEQ ID NO: 459 - DNA, 20 bp, Artificial sequence
  Synthetic oligonucleotide
caccccttctacactgcgag

SEQ ID NO: 460 - DNA, 20 bp, Artificial sequence
  Synthetic oligonucleotide
aaccctaccccaatttaccc

SEQ ID NO: 461 - DNA, 20 bp, Artificial sequence
  Synthetic oligonucleotide
acaggtggcattctacccta

SEQ ID NO: 462 - DNA, 20 bp, Artificial sequence
  Synthetic oligonucleotide
gcctactagacccctcttat

SEQ ID NO: 463 - DNA, 20 bp, Artificial sequence
  Synthetic oligonucleotide
gtataccaacttcaccatcc

SEQ ID NO: 464 - DNA, 20 bp, Artificial sequence
  Synthetic oligonucleotide
gtccacgaattcagtttgtg

SEQ ID NO: 465 - DNA, 20 bp, Artificial sequence
  Synthetic oligonucleotide
tgtttatctgaattcgccat

SEQ ID NO: 466 - DNA, 20 bp, Artificial sequence
  Synthetic oligonucleotide
ctcgccaccagccatgcgat

SEQ ID NO: 467 - DNA, 20 bp, Artificial sequence
  Synthetic oligonucleotide
gcaggccccttaagatctgt

SEQ ID NO: 468 - DNA, 20 bp, Artificial sequence
  Synthetic oligonucleotide
agtcttgataccactttagc

SEQ ID NO: 469 - DNA, 20 bp, Artificial sequence
  Synthetic oligonucleotide
gcaacaaccactaagacttg

SEQ ID NO: 470 - DNA, 20 bp, Artificial sequence
  Synthetic oligonucleotide
gcttgtttcctaaggcttgc

SEQ ID NO: 471 - DNA, 20 bp, Artificial sequence
  Synthetic oligonucleotide
agtttcactcacggattagg

SEQ ID NO: 472 - DNA, 20 bp, Artificial sequence
  Synthetic oligonucleotide
ccccgctgaaaaattaagga

SEQ ID NO: 473 - DNA, 20 bp, Artificial sequence
  Synthetic oligonucleotide
ccctgttatcctatggcctc

SEQ ID NO: 474 - DNA, 20 bp, Artificial sequence
  Synthetic oligonucleotide
tcctacctaacccagcgagt

SEQ ID NO: 475 - DNA, 20 bp, Artificial sequence
  Synthetic oligonucleotide
ccaagcctagatatcctatc

SEQ ID NO: 476 - DNA, 20 bp, Artificial sequence
  Synthetic oligonucleotide
ggcacataaaatgcagagca

SEQ ID NO: 477 - DNA, 20 bp, Artificial sequence
  Synthetic oligonucleotide
gagtattttgcaatgtcacc

SEQ ID NO: 478 - DNA, 20 bp, Artificial sequence
  Synthetic oligonucleotide
ggagtattttgcaatgtcac

SEQ ID NO: 479 - DNA, 20 bp, Artificial sequence
  Synthetic oligonucleotide
gcggagtattttgcaatgtc

SEQ ID NO: 480 - DNA, 20 bp, Artificial sequence
  Synthetic oligonucleotide
gtgcatccatccagtttctc

SEQ ID NO: 481 - DNA, 20 bp, Artificial sequence
  Synthetic oligonucleotide
cctggttatttcccatgagc